European Patent Specification EP 3 149 027 B1, published December 24, 2025. Title: AUGMENTATION DE LA RECOMBINAISON MEIOTIQUE CHEZ LES PLANTES PAR INHIBITION D'UNE PROTEINE RECQ4 OU TOP3A DU COMPLEXE RTR. Applicant: INSTITUT NATIONAL DE LA RECHERCHE AGRONOMIQUE. The sequence listing filed with the application follows.

SEQUENCE LISTING (46 sequences)

SEQ ID NO: 1 - protein, 1188 aa, Arabidopsis thaliana
MINSNQMSRSHLPEVQKPRGPQTNWSEHAKALESSSSVTKFLSSNVLYALESQKPRDMAARSIAFPSVNVHTLAHPQISKAWRALSSLSVNNTYLRPGVTPPIDVGTNDSYSARERSTAKVISSTGGSVYSSTRPNLSAMNVSGTGRSFHSFPSSVPGDDKIVAEKFPRGNNEIRESEPSCTHLNGVEKSFGNSAFPAEQFESRKACLDDMDDDDILENIDVDQIVMEHYHSTSTPQPSVSNFSLRTPPVDRSASRLEEECNLPPELCSNCSHGIKLGLCPEASTHVEQMKDVLLAISNELLDDATDLSPDRVGQLRQERLRLKKQIQQLENHIRDKESQKSQFLSSTATRIFQYETPKSTNYKMDQPQTDFRAHVSDQGRYACDSWNTPRDSSFSVDRYGLSSAPVEREQYVPKIIDVTYTEGSNDKKWSSREFPWTRKLEVNNKKVFGNHSFRPNQREIINATMSGSDVFVLMPTGGGKSLTYQLPALICGGITLVISPLVSLIQDQIMNLLQANIPAASLSAGMEWAEQLKIFQELNSEHSKYKLLYVTPEKVAKSDSLLRHLENLNSRGLLARFVIDEAHCVSQWGHDFRPDYQSLGILKQKFPNIPVLALTATATASVKEDVVQALGLVNCVVFRQSFNRPNLWYSVVPKTKKCLEDIDKFIKENHFDECGIIYCLSRMDCEKVSERLQEFGHKAAFYHGSMEPEQRAFIQTQWSKDEINIICATVAFGMGINKPDVRFVIHHSLPKSIEGYHQECGRAGRDGQRSSCVLYYGYGDYIRVKHMISQGGVDQSPMATGYNRVASSGRLLETNTENLLRMVRYCENEVECRRFLQLVHLGEKFDSTNCKKTCDNCCSSQSLIDKDVTLITRQLVELVKQTGERFSSAHILEVYRGSLNQMVKKHRHETLQFHGAGKHLSKIEVSRILHYLVTEDILVEDVRKSDMYGSVSSLLQVNNAKATILFSGSQTIVMKFPSSVKVLKPSKQGATAAKGPLTSEKQSTLPLTTEDAPPKDVNLSANMYTALRKLRTALVKEAPDGVMAYHIFINSTLQQISRRIPRTKEELLEINGLGKAKVSKYGDQLLETIETTVNEYYGTNKKDSIISNDSPDSGKRRRDENISPNVAEDDDFEVSPSQSCKKTVRNKSNEVLHGECIDGDRRGMELDFDFKDEDGSEIRPEGRVLPW

SEQ ID NO: 2 - protein, 926 aa, Arabidopsis thaliana
MSRRGGGPVTVLNVAEKPSVAKSVAGILSRGTFRTREGRSRYNKIFEFDYAINGQPCRMLMTSVIGHLMELEFADRYRKWHSCDPADLYQAPVMKHVPEDKKDIKKTLEEEARKSDWLVLWLDCDREGENIAFEVVDVCRAVKHNLFIRRAHFSALIDRDIHEAVQNLRDPNQLFAEAVDARQEIDLRIGASFTRFQTMLLRDRFAIDSTGEERSRVISYGPCQFPTLGFIVERYWEIQAHEPEEFWTINCSHQSEEGLATFNWMRGHLFDYASAVILYEMCVEEPTATVMNVPHPRERFKYPPYPLNTIELEKRASRYFRLSSEHTMKVAEELYQAGFISYPRTETDSFSSRTDLRAMVEEQTRHPAWGSYAQRLLEPEGGLWRNPANGGHDDKAHPPIHPTKFSSGESNWSRDHLNVYELVVRHYLACVSQPAVAAETTVEIDIAGERFSASGRAILAKNYLEVYRFESWGGSVIPVYEKGQQFIPTTLTLDAAVTRPPPLLCEADLLSCMDKAGIGTDATMHDHIKKLLDRGYATKDANTRFSPTNLGEALVMGYDDMGYELWKPNLRALMEHDMNEVSVGRKTKAEVLETCLQQMKACFLDARVKKSKLLEAMTIFFERSNNTDESESQTAGEVVRRCNLCNESDMALRKNRDGNFMVGCMNYPQCRNAVWLPGPTLEASVTTNVCQSCGPGPVYKILFKFRQIGIPPGFDVNHLGCVGGCDDILKQLIDICGTGSRSQARRTPGTAPSNNIQGSNTRQSNVCIHCQQRGHASTNCPSRVPASRNSRPTATNPRNDESTVSCNTCGSQCVLRTANTEANRGRQFFSCPTQGCSFFAWEDSINNSSGNATTGSNSGGSGRRGSRGRGRGGRGGQSSGGRRGSGTSFVSATGEPVSGIRCFSCGDPSHFANACPNRNNSNGNYF

SEQ ID NO: 3 - protein, 1189 aa, Arabidopsis lyrata
MSWSHLPEVQKPRGPQTNWSEHAKALESSSSVTKFLSSNVLYALESQKPRDMSARSIAFPSVNVHTLAHPQISKAWRALSSLSINNAYLRPGVTPPIDDGGTNGSYSAREGSTVKVISSTGGSVYSSSRQNQNAMNVSGTGRSFHSFPSSVLGADKMIAEKFPLGNDEVRESEPSFTHLNGVEKSFRNSAFPPEQFESGKACLGDMDDDDILKNIDVDQIVMEHYHSTSTPQPSVSNFSLRTPPAPPVDRSASRLEEECYLPPELCSNCSHGIKLGLCPEASTHVEQMKDVLLAISNELLDDAADLSPYRVEQLRQERLQLKKQIQQLENHIRDKERQKSQFSSSTATRTFQYETPKSTNYKMDQPQTDFRAHLSDQGRYAGDSWNTPRDSSFSVDRYGLSTAPVEREPYVPKIIDVTYTEGSNDKKWSSREFPWTRKLEVNNKKVFGNHSFRPNQREIINATMSGSDVFVLMPTGGGKSLTYQLPALICGGITLVISPLVSLIQDQIMNLLQANIPAASLSAGMEWAEQLKIFQELNSEHSKYKLLYVTPEKVAKSDSLLRHLENLNSRGLLARFVIDEAHCVSQWGHDFRPDYQSLGILKQKFPNIPVLALTATATASVKEDVVQALGLVNCVVFRQSFNRPNLWYSVVPKTKKCLEDIDKFIKENHFDECGIIYCLSRMDCEKVSERLQEFGHKTAFYHGSMEPEQRAFIQTQWSKDEINIICATVAFGMGINKPDVRFVIHHSLPKSIEGYHQECGRAGRDGQRSSCVLYYGYGDYIRVKHMISQGGVDQSPMATGYNRVASLGRILETNTENLLRMVSYCENEVECRRFLQLVHFGEKFDSTNCKKTCDNCCSSQSLIDKDVTLITRQLVELVKQTGERFSSAHILEVYRGSLNQMVKKHRHETLQLHGVGKHLSKIEVSRILHYLVTEDILVEDVRKSDMYGSVSSLLKVNNAKATLLFSGSQTIMMKFPSSVKVLKPSKQGATAAKGPLTSEKQSTLPLTTEDAPPKDLNLSANMYTALRKLRTALVKEAPDGVMAYHIFINSTLQQISRRIPRTKEELLEINGLGKAKVSKYGDRLLETIETTVNEYYGTNKKDSIISNDSPDSGKRRRDENISPNVAEDDDFEVSPSQSCKKTVRNKSNEVLHGECVDGDRRGMVMEKLDFDFRDEDVSEIRPEGRVLPW

SEQ ID NO: 4 - protein, 1172 aa, Arabidopsis lyrata
MTLIVKFVVEQHCSFHSDNRSQLKFVNGGDKRRSNCWKLFGIGSHLPEVNKSRGHFLQTNWSKHAKAFECIPSLNKFMGSNFLYSLESQKLARDREMGARSIENIAPVTVQTLARPEIEKAWCTLINLSINNTYLRPGITPAIDDGSTDRSSSTKRSTVKVTSSADGSFYAHNHPEHSQRSLRGTAKSFDSFSSSSVGDNNITIGKVPRVNDEVRDSVTGCKYTNGMEMPPIKNSAHLVRLVEPREASLGEIDYDDIMEIIEVDQIVMDHCPSRCPKQPSVSKFVDTFASRREEEQGLFPELCSNCSHGIKLGLCPEASTHVEQMKDTLLAISNEFLDNTYDLGPDHVEQLRQKRLLLKKQIQQLEILIQNKERKKSECLVSTPSHNIQYETPQTTNHVVVYTQTDSPDKSCGGLCPATEGRYVTDNWNMPRDYLVSKERYDISSGSVEREQSVSEVIDVTDTESSNDKKWASRDFPWTKNLEVYNKIVFGNHSFRPNQREIINATMSGCDVFVLMPTGGGKSLTYQLPALLCAGITLVISPLVSLIQDQIMNLLQTNISAASLSAGMEWAEQLEILQELSSENSKYKLLYVTPEKVAKSESLIRHLEILNSRSLLARFVIDEAHCVSQWGHDFRPDYQGLGVLKQKFPNIPMLALTATATTSVKEDVVQALGLVNCVVFRQSFNRPNLWYSVVPKTNKCLEDIDKFIRENHFDECGIIYCLSRMDCEKVTEMLRAFGHKAAFYHGSMDPGKRAFVQKQWSKDEINIICATVAFGMGINKPDVRFVIHHSLPKSIEGYHQECGRAGRDGQRSSCVLYYSYTDYIRVKHMISQGGLGQGQMKMGYNCKASSGRMLETNTENLLRMVSYCENEVDCRRFLQLVHLGEKFDSTNCKKTCDNCSSSKILIDKDVTVIARQLVELVKLTGERFSSAHIVEIYRGSLNQSVKRNRQETLHLHGAGKHLTKSEASRILHYLVTEDILAEGVRKSDLYGSVSSLLKVNRSKAASLLSGGQSITMRFPSTIKASKPSKSTAKVPLKQTTLPMAKAAPQDSNLPHILLTALKKLRSDIVKESSDGVMAYHIFGKATLEQISKRLPRTKEELLDINGLGKAKVSKYGDRLLETIYSTINDHYKTGPGSGKRRRDENICPNVADDDDPDWTASQSHKKAVKNKK

SEQ ID NO: 5 - protein, 1150 aa, Arabidopsis thaliana
MVVTRGDKFAGSSLACKSMIGANKMSGSHLHEVNNSRSHFPQTNWLKVAKAFECIPSLNKFMGSNFLYSLESQKLGRDREMAARSIENIAPVTVQTLARPQIEKAWCTLINLSINNTYLRPGITPAIDNDSTSRTSSTKGSTFKVTSNADGSFCAHNHPEHSQRSVRGTAKSIDSFSSSSVGDNKIIIDKVPRVNYEVRDSVTVTNGMEMPPIKNSAQLARPVEPREVSLGEIDYDDIMEIIDVDQIAMEHCPSTCTKQPSVSKFVDIFTSRREEEQGLPPEICSNCSHGIKLGLCPEASTHVEQMKDTLLAISNEILDNTYDLGPDHVEQLHQKRLLLKKQIQQLEILIHNKERKKSQCLVSIPSHNTQYETPQTTNLEVVYGQTDSPTHVKEQGRCVTDNWNMPRDYLVSKERYDISSGSEEREQSVSEVIDVTDTESSNDKKWTSSDFPWTKNLEVYNKLVFGNHSFRPNQREIINATMSGCDVFVLMPTGGGKSLTYQLPALLCAGITLVISPLVSLIQDQIMNLLQTNISAASLSAGMEWAEQLEILQELSSEKSKYKLLYVTPEKVAKSESLLRHLEILNSRSLLARFVIDEAHCVSQWGHDFRPDYQGLGVLKQKFPNIPMLALTATATTSVKEDVVQALGLVNCVVFRQSFNRPNLWYSVVPKTNKCLEDIDKFIRENHFDECGIIYCLSRMDCEKVTEALRVFGHKAAFYHGSMDPGKRAFVQKQWSKDEINIICATVAFGMGINKPDVRFVIHHSLPKSIEGYHQECGRAGRDGQRSSCVLYYSYTDYIRVKHMISQGGLGQGQMKMGYNCKASSGRMLETNTENLLRMVSYCENEVDCRRFLQLVHLGEKFDSTNCKNTCDNCSSSKILIDKDVTVIARQLVALVKLTGERFSSAHIVEIYRGSLNQSVKRNRQDTLHLHGAGKHLTKSEASRILHYLVTEDILAEGVKKSELYGSVSSLLKVNRSKAASLLSGGQSITMRFPSTIKVSKQSKSTANPAKVPLKQTTLPMAKAAPQDSNLSGILLTALKNLRTDIVKESPDLVMAYHIFGNATLKEISKRLPRTKEELLDINGLGKAKVSKYGDRLLETIDSTINDHYKTRPGSGKRRRDENVNPNVAEDDDPDWSASQSHKKVVKNKK

SEQ ID NO: 6 - protein, 1222 aa, Brachypodium distachyon
MQGSNKLNAGSSCNDKLPRVNWPHHASAIQSSSSKDDFLSSSFLFSLPTQRPNPEANCNSMISLRSAACKIQGPERLQVPWIEKVWTLLWQAWRSVCNTQVACKSYLRPGLSAKVEDCAKDYTHTYATNSSYNTNRQDNVPRNMIPSQEGIHQRTESGILENNSSHGPTGINSCTRTYQSNHVVRADNIGTTNHCGFARTDAKSCQNVPVADNMCADDTLDAMDDDEIMASIDVDRIVMEHYEATNTHRGLASWQMSTPSGNKCNLTGLDENSLPQELSEICIHGCKLAFCPEAKYHVQEMKDQMLAICSELIDGSGELSPQDSEALRKQRAHLKKQTKLLEDYMARSTQDDERQRSHSMATASQGHHPPMTPSTSVMDNDRFQSQIYSRNEPVNSGSCYPPAPHPYMDSLNTPLTSVQRDYTRTNIDINYTEGSGDKKWSSKDFPWTKELEAHNKRVFGNHSFRPNQREIINATMYGSDVFVLMPTGGGKSLTYQLPALIDEGITLVVCPLVSLIQDQIMHLAQANIPAICLSANVEWTEQQRILRDLMSPSSTCTYKLLYVTPEKIAKSDALLRQLEILYSRGHLSRIVIDEAHCVSQWGHDFRPDYQHLGLLKQKFPETPVLALTATATASVKEDVVQALGLANCVVFRQSFNRPNLRYIVMPKTKKCLEDIDNFIRASHHKECGIIYCLSRMDCEKVAAKLREYGHKASHYHGSMDPLDRTEIQRQWSRDKINIICATVAFGMGINKPDVRFVIHHSLPKSIEGYHQECGRAGRDGQRSSCVLYYNYSDYIRVKHMITQGVVEQETSMPRGGSLSSHRQALETHKENLLCMVSYCENDVDCRRLLQLIHFGETFDPSCCAKTCDNCMKEMRWIEKDVTTIARQLVELVMMTRPACSTSHILEVFRGSVNQNVKKNRHDTLSLHGGGKNLAKGEASRVLRHLVTEGILIEDVKKSDTYGLVSSVLKVNQMKVGGLRSGNHTIVLKFPTREAPLMGKLDESSTPQINKTAQRQSEVDENISSLLFETLKCLRSQIAESTAGCGVHHIFKNETLKEISSRVPRTKEELLEINGIGKVKLNKYGDSVLATIEDFLSHFPNASKRSSSSGSNEQNEAPKKRRGLSATNASGKCDGFEERTVQSKKCAAKTKNTKQGISDAASMVQDVRYIDLDLDGCEDVDDELCSSAQQPVASSRVLPKWPTAVTKGNSPVANLFEEFKYTK

SEQ ID NO: 7 - protein, 1162 aa, Brassica rapa
MSLSEVQKPKAPQTNWSEHVKVLDGSPSSVTKHLSSNFLYALESQKPGRCRDMAARSIAFPSVNVHTLAHPQIAKAWRALSSLSINKTYLRPGITPPVDDSGTNGSYSARESSTVKVTSSTGGSFYSNNQQNQSQMGVPGTGRYSHSFPSSVPGDDKRAAEKFSRVNDEVREPETSCAHSNGVEKPFRKSALAAEQLESGEACLDEINDDILQNIDVDQILMEHYQSTSTPQPSVSSFPLRTPPVDRSASSREEEFCLPPELCCNCSHGIKLGLCPEASTHLEQMKNTLIAISNELLDDDTDLSPDRIQELRQERLQLKKQIQQLENHIRDKERETSKFLSSTATPFQYETPKATNRNMDDPQTDSRAEFSEQGGYASGSWNMPRDSSFSVDRYGLSSAPVEREQYVPRIIDVKYTEGSSDKKWSSREFSWTKKLEVSNKKVFGNHSFRPNQREIINATMSGSDVFVLMPTGGGKSLTYQLPALICQGITLVISPLVSLIQDQIMNLLQANIPAASLSAGMEWAEQLKIFQELSSEHSKYKLLYVTPEKVAQSDSLLRHLDSLNSRGLLARFVIDEAHCVSQWGHDFRPDYQSLGILKQKFPNIPVLALTATATASVKEDVVQALGLVNCVVFRQSFNRPNLWYSVVPKTKKCLEDIDKFIRENHFDECGIIYCLSRMDCEKVAEKLKEFGHKAAFYHGSIEPTQRALVQKQWSKDEINIICATVAFGMGINKPDVRFVIHHSLPKSIEGYHQECGRAGRDGQRASCVLYYGYGDYIRVKHMISQGGVDQSPMAGGYNRVASSARLLETNSENLHRMLRYCENEVDCRRFLQLVHFGEKFDSTNCKNTCDNCCSSQSLIDKDVTLITRQLVELVKQTGERFSSSHILEVYRGSLNQMVKKHRHETLQFHGAGKQLSKIEVSRILHYLVTEDILVEDVRKSDMYGSVSSLLKVNNAKAASLFSGSQTIMMRFPSSVKVLKTTKPAPTPAKAPVTSADTPPEDLNLSAIMYTALRKLRTLLVKEAPDGVMAYHIFGNATLQQISKKIPRTKEELLEINGLGKAKVTKYGDRLLETIESTVNEYYGTSNKDSMISPDTGKRRRDENTSPNVADDDDDFAEMSIQSCKKTARNKSNEIGMVVEKLDFDFEDEDGSELRPEGRVLPW

SEQ ID NO: 8 - protein, 1159 aa, Brassica rapa
MVVVTRDDRLAGALPHVQPMSAANKMCGSHLPEAQKSRVHLPQTNWLKHANAFECIPSSNNFLSSSMLYSLESQKPSRSRETASRPIYNIIPVDVQTLAHQHISKAWCALANLSINNTYLRPGITPAIDDINTNCSFSTRGRSTAKVTSNTDGSFFAHNHQEDSQKRIRGTATSFDRFSSSSPGDGKLISGKVPRVYNEVRDSVTGCINGMEVPPIRNLAHPARQVEVIEIDDDDILKSIDVEKIVMEHYHSTCTHQPSVNIFASRGEENPCLPPELCSNYSHGVKLGLCLQAPSHVEQMKDALLAVSNELLDDSTDLSPGHFEQLCQERLLLKKQIQQLEILIQDKEKKSSGCLASRPTRNIQYETPQTTNRKADYAHADSRVHVTEQGRYVSDNWNMPRDYLCSEDRSGLSSGPIERERCVPEIIDVTYTDGSNDKKWSSRDFPWTKNLEVNNKRVFGNHSFRPNQREIINATMSGCDVFVLMPTGGGKSLTYQLPALICAGITLVISPLVSLIQDQIMNLLQANIHAASLSAGMDWTQQLDILRELSSENSKYRLLYVTPEKVAKSDSLLRHLESLNSHSLLARFVIDEAHCVSQWGHDFRPDYQGLGILKKKFPKIPMLALTATATASVKEDVVQALGLVNTVVFRQSFNRPNLWYSVVPKTNKCLEDIDQFIKKNHFDECGIIYCLSKMDCEKVTETLRKFGHKAAFYHGSMDPGKRAFVQKKWSKDEINIICATVAFGMGINKPDVRFVIHHSLPKSIEGYYQECGRAGRDGQRSSCVLYYCYSDYIRVKHMISQGGPGQSTMTTGYNRIASSGRTLESNTDNLLRMVSYCENEVDCRRFLQLVHLGENFDSTNCKNTCDNCSSSKTLIEKDVTLIGRQLVELVKLTGERFSSAHIVELYRGSLNQTVKKHRHETLHLHGAGKHLSKSEASRILHYLVTKDILTEYVKKSDLYGSVSSLLKVNRSKAASILSGGQTIEMRFPSAVKAVKPSKQGPTPARVALKQTTLPMAPAPPQDSILSDTLVKALKNLRADIVKESSDAVMSYHIFGNPTLQQISKRLPRTKEELLDIHGLGKAKVSKYGDRLLETIESTINNHYGTNKNEGTGSGKRRRDENTNPIVVDNDDDDPDWTPSQQSYKKAYAVRGQTSEEAIC

SEQ ID NO: 9 - protein, 1196 aa, Brassica rapa
MINSDQVSRSHLPEVQKPKAPQTNWSEHANAFEDPSSRTKHLSSGFLYALESQKPRKSSDMAARSIAFPSVNAHTLAPPQIAKAWRALSSLSLNKTYLRPGITPPVDDGGTNGSYSARERSTVKVTCSTDGSFYSNNQQNQSQMGVPGTGRSFHSFPPPVPGDGKNFAEKFRRINDETREPETSSAHLNGVEKPFKNSTFAAEQLGSGEACLDEIDDDILQNIDVDQIMMEHYQSTSTPPSSVSSLPSRTPPVDRSASRREEECSLPPELCSNCSHGIKLGLCPEASTHLEQMKNMLIAISNELLDDDTDLSPDRIQELRQERLLLKKQIQQLEDHIRDKEKQKSQFLSSTATRASQYETPKSTNLRFDHPQTDSRAHFNEQGRYASDSWNMPKDSSFSVDRYGLSSAPVEREQYVPRIIEVTYTEGSNDQKWSSRDFPWTRKLEVSNKKVFGNHSFRPNQREIINATMSGSDVFVLMPTGGGKSLTYQLPALICQGITLVISPLVSLIQDQIMNLLQANIPATSLSAGMEWSEQLKIFQELSSEHSKYKLLYVTPEKVAQSDSLLRHLDNLNSRGLLARFVIDEAHCVSQWGHDFRPDYQSLGILKQKFPNIPVLALTATATASVKEDVVQALGLVNCVVFRQSFNRPNLLYSVVPKTKKCLEDIDKFIKENHFDECGIIYCLSRNDCEKVAQKLQEFGHKAAFYHGSIEPTQRALVQKQWSKDEVNIICATVAFGMGINKPDVRFVIHHSLPKSIEGYHQECGRAGRDGQRASCVLYYGYGDYIRVKHMISQVGVEQSPMANGYNRVASSGRLLETNTENLLRMVRYCENEVDCRRFLQLVHFGEKFDSTNCKRTCDNCSSSQSLIDKDVTLITRQLVELVKQTGERFSSSHILEVYRGSLNQMVKKHRHETLQFHGAGKHLTKLEVSRILHYLVTEDILVEDVRKSDMYGSVSSLLKVNKSKAASLFSGSQTIMMRFDFVLEIYLSSKRFPSSVKVLKPCKAAPTPAKAPLVSADAPPEDVNLSAIMYTALRKLRTLLVKEAPDGVMAYHIFGNATLQQMSKKIPRTKEELLEINGLGKAKVLKYGERLLETIESTVNEYYGTSKKEESMISPDSGKRRRDENISPNVTEEDDDFAESSSQSCKKTVRSKSSEVLHGECVAGDGVGMVMEKLDFDFEDEDGSEIRPEGRVLPW

SEQ ID NO: 10 - protein, 963 aa, Carica papaya
MTNFLKVLSSNFLFSLEKQKPSTEGRTGARSVACQIKNLQRLRSPQSEKAWQILSNPPTGRTYIKPGLTASLKHDIDNSLDGIRKTSLQTTYGSSKNSKYTHTRRNCSQINAKTTETAKYMDSCPPDIVDTTETRTGLRVHNKVDALVSNGTHSNALDGSYGDRPMHAGQTKERPEVSADGMDDDDILKNIDVDQIVMEHYQSTCTPQPSISMFPPRMPNVERNSSAREEESCLPPELCSKCIHGFKVGVCPEACTHVQEIKDQLIAISNELLDNAAELTKEQLEELRQDRLRLNKQLQQLETYLCDMERKRSHFSTSATTHSSQYDTPQARIFRMDHLGSGDQFHLNESHIHMKWNPYSESISSEGRVAISSGNVERELYIPKVIEVNYIEGSNDHKWSSRDFLWTKKLEINNKKVFGNHSFRPNQREVINATMSGYDVFVLMPTGGGKSLTYQLPALICPGITLVISPLVSLIQDQIMSLLQANIPATYLSANMEWAEQLEILKELSSDYCKFKLLYVTPEKVAKSDVLLRHLEGLNARGFLSRIVIDEAHCVSQWGHDFRPDYQGLGILKQKFSNTPVLALTATATASVKEDVVQALGLVNCIVFRQSFNRPNLWYAVVPKTKKCLEEINKFVKENHFDECGIIYCLSRMDCEKVAEKMQEYGHKAAFYHGSMDPAQRSFVQEQWSKYEINIICATVAFGMGINKPDVRFVIHHSLPKSIEGYHQECGRAGRDGQRSSCVLYYSYSDYIRVKHMISQGVAEQGTLTPGYNRMANSGRILETNTENLLRMVSYCENDVDCRRFLQLGHLGEKFDHANCKRTCDNCSKNKSLIEKDVTKTAKQLVELVKLTGQQFSSSHILEVYRGSLSKYVKKHRHETLSLHGAGKLLTKEEASRVLRHLVTNDILVEDVKKSDIYGSLSSVLKVNESKAYNLFSDGQTITLRLNFMLKLLLSNLIMNVQH

SEQ ID NO: 11 - protein, 1170 aa, Thellungiella halophila
MINSNQIRSHLPEVQKPKGPQTNWSEHAKALESTSFLSSNFLYDLESQKPRRDRDMAARAIAFPNVNVHTLAHPQIAKAWRALSSLSVNNSYLRPGITPPVDDGATNGSYSAKERSTVKVTCSTDGSFYPNSRQNQSHMSVSGTGRHFHSSSAPGEEKFVAEKFARVNGEVRESETSSTHLNGLENPFRNSAFPDEQLESGEAFLDDDDILMNIDLDQIAMEHYQSTSTQPSVSNFPLRNPPVDRSASRREEECLPPELCFNCSHGIKLGLCPEASTHLEQMKNVLIAVSNELLDDDTDLSPDRAKQLRQERLQLKKQIQQLENHIRDKERQKPQSLSSAPTPGFQFETPKSTNRKMDLPQTEFQAHLSEQGRYACDSWNMPRDSSFSVDRYGLSSAPVEREQYVPRIIDVTYTEGSNDKKWSSSDFPWTRKLEVSNKKVFGNHSFRPNQREIINATMSGSDVFVLMPTGGGKSLTYQLPALICKGITLVISPLVSLIQDQIMNLLQANIPAASLSAGMEWAEQLKIFQELSSEHSKYKLLYVTPEKVAKSDSLLRHLESLNSRGLLARFVIDEAHCVSQWGHDFRPDYQSLGILKQKFPNIPVLALTATATASVKEDVVQALGLVNCVVFRQSFNRPNLWYSVVPKTKKCLEDIDKFIKENHFDECGIIYCLSRMDCEKVAEKLQDFGHKAAFYHGSIEPAQRALVQKQWSKDEINIICATVAFGMGINKPDVRFVIHHSLPKSIEGYHQECGRAGRDGQRSSCVLYYGYGDYIRVKHMISQGGVDQSPMASGYNRVASSGRILETNTENLLRMVSYCENEVDCRRFLQLVHFGEKFDSTNCKKTCDNCCSSQSLIDKDVTLITKQLVELVKQTGERFSSSHILEVYRGSLNQMVKKHRHETLQLHGAGKHLSKIEVSRIMHYLVTEDILVEDVRKSDMYGTVSSLLKVNHSKAASLFSGSQTIMMRFPSSGKVLKPSKPAATPAKGPITSAADAPPEDLNLSVRMYTALRKLRTLLVKEAPDGVMAYHIFGNATLQQMSKKIPRTKEELLEISGLGKAKVSKYGDRLLETIESTVSEYYGTNKKDSVINNDSPDSGKRRRDENISPNVAGDDDFAESSTQACKKAVRNKSNEARRGENVDGYGVGMVMDKLDFDFEDEDGSEIRPEGR

SEQ ID NO: 12 - protein, 1148 aa, Thellungiella halophila
MVVTREDKFAGSYLGVKPMIGPYKLRQNCGSYLPEVENSRGHFPQTNWSEHAKAFECIPSVNKSLSSNLLYSLESQKHRRSRDSASRPIENVIPVNMQNLTRQQIEKAWCALTNLSINHTYLRPGITPAVDDSSTNCTSSMRGRSTVKVTSNADGSFYAHNHPEQSQESVRGTARSFDRFSSSFPGDGKLTAGKVPRVNNEVRDSVTGCKYINGMDIQPIRNFALPARQVEASLIEIDDDDILEIIDVDQIVMENYHLTYTPQPSVNIFASRGEEVPCLPPELCSNCSHGVKLGLCLEASTHVEQMKDALLAISNKLLDDSTDLSRDHSEQLCQERLLLKNQIQQLEILIQNKERKKSSTPTHNFQYGTPQITNCKVDYAQTDSREEQGRYVSDNWNMPRDYLLSEDRYGLSSGPVERERHVPEIIDVTYTDGSNDTKWCSRDFPWTKNLEINNKRVFGNHSFRPNQREIINATMSGCDVFVLMPTGGGKSLTYQLPALICAGITLVISPLVSLIQDQIMNLLQTNIPAASLSAGMEWGEQQEILRELSSGNSKYKFLYVTPEKVAKSDSLLRHLESLNSHSLLARFVIDEAHCVSQWGHDFRPDYQGLGVLKKKFPNIPMLALTATATASVKEDVVQALGLVNCVVFRQSFNRPNLWYSVVPKTNKCLEDIDKFIRENHFDESGIIYCLSRMDCEKVTEALQKFGHKAAFYHGSMDPAQRAFVQKQWSKDEINIICATVAFGMGINKPDVRFVIHHSLPKSIEGYHQECGRAGRDGQSSSCVLYYSYSDYIRVKHMISQGGPGQGPTTMGYNRLASAGRILETNTENLLRMVSYCENEVDCRRFLQLVHLGETFDSTNCKKTCDNCSSSRSLIDKDVTLIARQLVALVKLTGERFSSAHIIEIYRGSLNQTVKKHRHETLHLHGAGKHLAKSEASRILHYLVTKDILAEYVKKSYLYGSVSSLLKVNRSKADAILSGGQTIIMRFPSAVKVSKTSKSGAIPAKAPLKQTTFTPLMTHAPSQDSILSVTLYTALKKLRTDIVKESSDAVMAHHIFGNGTLRQISKRLPRTKEELLDITGLGKAKVNKHGDRLLEIIESTINEHYRTEKSEGPGSGKRRRNENISPNVADDDDPDWTPTHSHKKAVKNK

SEQ ID NO: 13 - protein, 1202 aa, Eucalyptus grandis
MQTRRREGGDDRLPRVNWSDHASAHDDFSNQSKFLSSNFLYSLPNQRPPVQESMGSRSMVFSMVNPQRLPTNQIDKAWHALSSLRISSRTYITPGKTLPVKDDNAGHSNKVSRTVSSSGKEHGHSWESNKKLNKSTARIDASNNYVSNPVVLAHYEAAEGGCPARQSGNGILGANKAHSEGFAAAMNRDSMPNAQTKSSGGVLADELDDDDILESIDVDQIVMEHYQSTSTPQPSIQKLPPITPDVERNSLQQDESCLPEELRSNCSHGLKLGLCPDAARHLQEMKDNLIAISNELLDNVTELTPEAVEKLRHDRSHLNRQIQQLENHLRSLTVDEERRKSHFSASAAPPTSSLYETPRAFGSRVEPFRLEAHVHPQNEPGGYDRWNSPSVSFTSDRFPVSSGPVDRDSCIQKPVEVNYTEGSIDKKWSSWSFPWTKSLEDHNKKVFGNHSFRPNQREIINATMSRYDVFVLMPTGGGKSLTYQLPALICPGVTLVISPLVSLIQDQIMHLLQANIPATYLSANMDWSEQQEILRELNSDYCKFKLLYVTPEKVAKSDVLLRQLESLHARELLARIVIDEAHCVSQWGHDFRPDYQGLGILKQKFPSTPVLALTATATASVKEDVVRALALVNCIIFRQSFNRPNLRYSVIPKTKKCLEDIDKFIKENHFDECGIIYCLSRMDCEKVAEKLQEYGHKAAFYHGSMDPAQRAFVQKQWSKDEINIICATVAFGMGINKPDVRFVIHHSLPKSIEGYHQECGRAGRDGQHSSCVLYYSYSDYIRVKHMISQGAVEQSPFSNGYNRINMANSGRVLETNTDNLLRMVSYCENDVDCRRLLQLVHFGEKFDSNNCGKTCDNCLKIKSFVEKDVTEIAKQLVELVKLAGQQFSSAHLLEVYRGSLNQFVKKHRHEKLNLHGAGKHLAKGEASRVLRHLVTEDFLVEDVRKSDLYGSLSSILKVNESKAYNLCSGRQSVILRFPSVAKISKSSKSDVTPAKGLSTFGKLMPQIDGPAQTEAQGDLILSAKLYTSLRMLRTILVKEAGDGVMAYHIFGNATLQHISKRIPRTKEELLEINGIGKAKVSKYGDRLLETIETTIREYQGTDNRNSSSSNDSMDSMKRRREANGGTKPNYEEDDDFTRSTGRSKKRATVIEAQNYNNQAVNEPGDDITCIDDLDFEDYDFDVDVDASNVNSGGRVLPSWSKS

SEQ ID NO: 14 - protein, 1152 aa, Glycine max
MRHGEANSGQGPKVNLLQHANALENFSSQAKFLSSTFLFSVPPKKPHHEQPNPGFVFRRSETIQGSQRVQVEKALAAHSSLQNSSRNYVQPGKTQVTPQLHEDRRTTSFHGGYENGNHRCPDVAATPIVNNHNSRGLDGSVNNHTNYTGQINKSSNCMAVDIDDDDSLFKNIDVDQIVEDYCTPKPSISKLPPITPTADKDNFARQGDDVLPPELCLDCVHGYMLGFCPEAASHLQDMKDNLIAIFNELLDNGENLNSTQIAKLRHDRSQLNKQIQQLEKYIHSGNLNEERQKSHFSASTAPPTSFVYETPQQTVLCNGSKRYDTEAYMGNGTYGSSFQSLPPFSVDNCSMPSGSVGREVFIPKIIEVNYIEGSGDKRWSSYDFSWTKELEVNNKKVFGNHSFRPNQREIINASMSGCDVFVLMPTGGGKSLTYQLPALIHPGITLVISPLVSLIQDQIMHLLQANIPAAYLSANMEWTEQQDILRELNSDYCKYKLLYVTPEKVARSDNLLRHLDNLHFRELLARIVIDEAHCVSQWGHDFRPDYQGLGILKQKFPNTPVLALTATATASVKEDVVQALGLVNCIIFRQSFNRPNLRYSVIPKTKKCLEDIDKFIRENHFDECGIVYCLSRMDCEKVAEKLQECGHKCAFYHGSMDPVQRASVQKQWSKDEINIICATVAFGMGINKPDVRFVIHHSLPKSIEGYHQECGRAGRDGQHSSCVLYYTYSDYIRVKHMLSQGAIEQSSMTSGYNRSNMINSGRILETNTENLVRMVSYCENDVDCRRLLQLAHFGEKFNSSTCLKTCDNCLKITSFIEKDVTEIAKQLVELVKLTGQRFSSSHILEVYRGSLSQMVKKHRHESVSLHGAGKHLAKGEASRILHHLVVEDFLWEEVKKSDFYGSVSSILKVNEPKIHNLFAGQRIILRFPSLVKASKPGKSDATPAKGSLTSGKLNVMQIDPPSPQTEVDDILSAKLYNALRLLRKSLVTEAGDGVMPHHIFGNATLLLISKRVPRRKEELLDINGIGKAKVSKYGDQLLESIEKTINEHYKLDKVSSGSKGSSDSTKKRRLSNGNPDANAEDDDAPTKSTGRSKKRMVKRQNRKAVIYDSPEEDYFQGCPDEDLDFDIIEIDALDQVTCKNAAGRVLPQWTAS

SEQ ID NO: 15 - protein, 1160 aa, Glycine max
MRQGEANSTQGPKVNLLQHANALENFSSQAKFLSSTFLFSVPPKKPPHHAEPNPGTAGFVFRRSETIQGSHRVQVEKALTAHSSLQNSSRIYVQLGKTQVTPQLHEDRRTTSFHGRYENDSRICPDVTVTPIVNNHSSRGLDGLVNNHTNYTGQIIKSSNCMAVDIDDDDDAILANIDVDQIVEEHQSTCTPKPSISKFPPITPTADKDNFARQGDNVLPPELCLDCIHGYKLGFCPEAASHLQEMKDNLIAISNELLDNGENLNSTQIAKLRHDRSQLNKQIQQLEKYIHSGNLNEERQKSHFSASTAPPTSFVYETPQQTVLCNGSKRYDTQAYMGNETYGSSFQSLPSFSVDNCNMPLGSVGREAFIPKIIEVNYIEGSGDKRWSSYDFPWTKELEVNNKKVFGNHSFRPNQREIINASMSGCDVFVLMPTGGGKSLTYQLPALIRPGITLVISPLVSLIQDQIMHLLQANIPAAYLSANMEWAEQQEILRELNSDYCKYKLLYVTPEKVARSDNLLRHLDNLHFRELLARIVIDEAHCVSQWGHDFRPDYQGLGILKQKFPNTPVLALTATATASVKEDVVQALGLVNCIIFRQSFNRPNLWYSVVPKTKKCLEDIDKFIRVNHFDECGIIYCLSRMDCEKVAEKLQECGHKCAFYHGSMDPAQRASVQKQWSKDEINIICATVAFGMGINKPDVRFVIHHSLPKSIEGYHQECGRAGRDGQRSSCILYYNYSDYIRVKHMLSQGAIEQSSMTSGYNRSNMINSGRILETNTENLVRMVSYCENDVDCRRLLQLAHFGEKFNSSTCQKTCDNCLKITSFIEKDVTEIANQLVELVKLTGQRFSSSHILEVYRGSLSQMVKKHRHETVSLHGAGKHLAKGEASRILHHLVVEDFLGEEVKKSDFYGSVSSILKVNEPKVRNLFAGQRIILRFPSSVKASKPGKSDATPAKGSLTSEKLNVMQIDPPSPQTEVDHILSAKLYNALRLLRKSLVTEAGEGVMPHHIFGNATLLLISKRVPRTKEELLDINGIGKAKVSKYGDQLLETIEKTVNEHYKLDNIGSGSKGSADSTKKRRVPNGNSDTNVEDDDAPTKSTGRSKKRTVKRQNRKGVIYDSPEEDYFQGCPDEDLDFDIIEIDALDQVTCKNTAGRVLPQWTAS

SEQ ID NO: 16 - protein, 1203 aa, Gossypium raimondii
MPDQSNSVESQKCYDKLPNVNWLQHFDAHDKFACQKKFLCTNFLFSLEGQKPQGTMFARLTSRQIQNSQIFQHTQVEKAWQILSSLPASCRTYLKPGTSAPVKTSTDEISHNRRGRSTLVEPSGMKRSEHMLVHPNSSETDGKVNGFGRCMTSSFPSNNANTMESGNNLRGNSGITTSMFSHSNSKVSGGSLKNQTFHGVQQEQSAEVLANEIDDDDLLKDIDVDQIVSEHYQSTCTPQPSVSKFPPITPSVDKNAFAGQETCLPPELCSNCSHGCKLGHCPEAASHVQEMKDMLIAVSNELLDNATNLSPEQIEKLRQDRLLLNKQIQLLEKYISDVERQKSNFSASTATLSFQYGTPQTTSLRPNLIQFDTQVHSRNEPNGYDNWNSPTVPFSSVNSFGVPSGPIEREPYIPQIIDVNYIEGSNDQKWSSRDFPWTRKLEANNKKVFGNHSFRPNQREVINATMSGYDVFVLMPTGGGKSLTYQLPALICPGITLVISPLVSLIQDQIMHLLQANIPAAYLSANMDWSEQQEILRELTSDYCKYKLLYVTPEKVARSDVLLRHLNILNSRDLLARIVIDEAHCVSQWGHDFRPDYQGLGILKQKFPKTPVLALTATATASVKEDVVQALGLINCIIFRQSFNRPNLWYSVIPKTKKCVEDIDKFIKENHFDECGIIYCLSRMDCEKVAEKLQEYGHKAAFYHGNMDPAQRAFIQKQWSKDEINIICATVAFGMGINKPDVRFVIHHSLPKSIEGYHQECGRAGRDGQRSSCLLYYSYSDYIRVKHMISQGAAEQSPLITGHSRFNNSGRILETNTENLLRMVSYCENDVDCRRLLQLLHFGEKFDSTHCQKTCDNCCKTSCSVDKDVTNIAKQLVELVKLTGQQFSSSHILEVYRGSLSQFVKKHRHETLSLHGVGKHLAKGEASRIIHHLVVEEYLLEDVKKSDIYGSVSSVLKVNESKVKNLFSGRQAIIIRFPSTVKVGKLSKPEVTPAKGSLTTSGKLSPPRVDTPAQFQSIVDLNLSAKLYSALRMLRTILVKEAGEGVMAYHIFGNATLQHISKRVPRTKEELLEINGIGKAKILKYGDRLLETIEATIKEHYKTDKINSGSSNDSNDSAKRRRNTNANIDNDDDFSRSTGRSKRRTVERQDKDGNGDNNHQYPADENDLDFDDLDYVYDVESKENRPQVEVNINGRMLPSWPRT

SEQ ID NO: 17 - protein, 1230 aa, Manihot esculenta
MRKNLSNSGQDNKCNEKLPEVNWSQHANAHDNFSSQKKFLSSNFLFSLEGQKPCIEGSMAMRLTCCQIQSLQRLQSQEVEKAWHTLCTLQISCRNYLQPGKTGPLKNARNDSLQDVGKPTLHSSSNRRKDSEDMHANQNFRDSSLRNNESTRYTGNVFPQDNARAAEAGSDMGRQNNIKGSAINNTQSKAFVGLMSNHIVHTKQSKESPEALADFIDDDDLLGNIDVDQIVMEHYQSTSTPQPSVSKFPPITPTADKNNFMRSEETFLPSELCQNCNHGFKLGLCPEAANHLQEMKDMLISVSNELLDNTANLSPAQIEKLRQDRLQLNKQIQQLEKYLCDGERQNSHFSASTATRNFQYETPQSAACRIDPPRFNAQFQLPNGPGGHENWNLPSVSFSSVDRFGLSSGPVDREPYIPKFIEVNYIEGSNDPKWSSTNFSWTKKLEAYNKKVFGNHSFRPNQREVINASMSGFDVFVLMPTGGGKSLTYQLPALISPGITLVISPLVSLIQDQIMHLLQANISATYLSANMDWTEQQEILRELCSDYCKYKLLYVTPEKVAKSDVLLRHLDSLNARGLLARIVIDEAHCVSQWGHDFRPDYKELGILKKKFGKTPVLALTATATASVKEDVVQALGLVDCIVFRQSFNRPNLWYSVIPKTKKCLDDIDQFIKGNHFDECGIIYCLSRMDCEKVAKKLQECGHKAAFYHGNMDSAQRAYIQKQWSKDEINIICATVAFGMGINKPDVRFVIHHSLPKSIEGYHQECGRAGRDGQRSSCVLYYSYSDYIRVKHMIIQGQIEQNPWTPGYNRTNMTNSERVLEKNTENVLRMVSYCENDVDCRRLLQLLHFGEKFDSGNCKKTCDNCSKIKTLVEKDVTEIAKQLVELVKLTGQQFSSSHILEVYRGSLNQYVKRYKHETLSLHGAGKHLAKGEASRILRHLVTEDFLVEDVKKSDIYGSVSSVLKVNESKAYNLCSSGQTIVLRFPSAVKVSKLSKYDATPAKGTLTYGEQSPLVDAPAQPQSEVDLSLSAKLYSALRMLRTILVKEAGDGVMAYHIFGNATLQHLCKRIPRTKEELLEINGIGKAKVSKYGDRLLETIESTIREHHNTDKNSSGSNDSTDSIKRRRDATRAAKLNVEEEDDFTKSTGRSKKRAAKLQNKDTEVYNARETDQNQCLDDDLDFEDSCYDHETNGSAVEADKNGTGRVLPSWSTPGNKIKSSNHNLFQEYAMNS

SEQ ID NO: 18 - protein, 1174 aa, Oryza sativa
MIKPRVNWSDHANAVQSSCIKDEFLSSSFLFSLPTQRPNQEADCTGMLPLRSAACRIQGLERLQAPSIEKAWRSLRNTQVARKNYLRPGLSGKVKDCDSDHAHTYGTSSSYNVNKMDSVSRNRNPTQESMHQTTESGTMEKNSSHLPAGTKSCTRTYLNNHVVQADTITTTNQSLARTGPELFKTAPFIDNMCDDAKLDAMDEDELLASIDVDRIVMEHYQATNTPRGSSKSPLEKCNFNGFDENNLPQELSIMCDHGSKLAFCPEAKSHLLEMKDNLLAISHELIDGQLSPQQSDDLHQKRALLKKQIELLGEYTARLTQDEERQQSHSMASTTAHQGHHPTSILSSSFVKDTNIFQSPIYTRNEPGESGLCFSSAPYSYMDGLSMPLPSVQRDYTPRAIDISYTEGSGDKQWSSTHFAWTKELEANNKRVFGNRSFRPNQREIINATMSGNDVFVLMPTGGGKSLTYQLPALICNGVTLVVSPLVSLIQDQIMHLLQANISAAYLSASMEWSEQQEILRELMSPTCTYKLLYVTPEKIAKSDALLRQLENLYSRGHLSRIVIDEAHCVSQWGHDFRPDYQHLGILKQKFPQTPVLALTATATASVKEDVVQVLGLANCIIFRQSFNRPNLRYFVWPKTKKCLEDIHNFIHANHNKECGIIYCLSRMDCEKVAAKLREYGHTASHYHGSMDPEDRANIQKQWSKDRINIICATVAFGMGINKPDVRFVIHHSLPKSIEGYHQECGRAGRDSQLSTCVLFYNYSDYIRLKHMVTQGFAEQGTSAPRGGSSQEQALETHKENLLRMVSYCENDVDCRRLLQLIHFGEMFNPSCCAKTCDNCLKELRWVEKDVTNIARQLVDLVMMTKQTYSTTHILEVYRGSVNQNVKKHRHDTLSLHGAGKHLAKGEAARILRHLVIEEILIEDVKKSENYGSVSSVLKTNHKKSGDLLSGKHNVVLKFPTPEKAPKMGVLDESSVPRINKTNQQSQVDGSLAAELYEALQCLRTQIMDENPQLLAYHIFKNETLKEISNRMPRTKEELVEINGIGKNKLNKYGDRVLATIEDFLARYPNATRKTSSGGSNEHSEAVKKRRGFSVTNTSTNCDDFEERTVQSKKRAAKTRTRQEISDAASIVQDVRYIDLELDGCEQVNEVPYSVQKPVASGRVLPAWQSARIA

SEQ ID NO: 19 - protein, 1167 aa, Phaseolus vulgaris
MCCLVGTQMRQGEANSVRVVKENNKNWLQHANAHENFSSQEKFLSSNFLLSVPPKKPRHQEPNPGTSGFVFQRSENIQVSQRVQFDKAWDVLSSLQNSSRTYIQPGKTVKVTRQIHENTRTTPFHGGYENDNRTCPDVTAAPVVSSHSSRGLDGSVNNHNKYTGQINESSNCMSGDIDDDNILENIDVDQIVEKYQSTCTPKPSISKLPPITPIADKDDFAREGDNALPPDLCLDCIHGYKLGLCPEAAIHLQELKDNLIAISNELLDNGENLNSTQISKLRHDRSQLNKQIQQLEKYIQSGNLNEERQKSHFSASTAPSTSYVYGTPQQTAPCNGSKRYDAQAYMGDGTFGSSFQSLPSFSIDKYSTLSGPVEREAFIPKIIEVNYIEGSGDKRWSSHDFSWTKELEVNNKKVFGNHSFRPNQREVINATMSGCDVFVLMPTGGGKSLTYQLPALICQGITLVISPLVSLIQDQIMHLLQANIPATYLSANMEWTEQQEILRELTSDYCKYKLLYVTPEKVVKSDNLLRHLENLHFRELLARIVIDEAHCVSQWGHDFRPDYQGLGILKQKFPNTPVLALTATATASVKEDVVQALGLVNCVIFRQSFNRPNLWYSVVPKTKKCLEDIDKFIRENHFDECGIIYCLSRMDCEKVAGNLQECGHKCAFYHGSMDPPQRAFVQNQWSKDEINIICATVAFGMGINKPDVRFVIHHSLPKSIEGYHQECGRAGRDGQRSSCVLYYSYSDYIRVKHMISQGGAIEQSPLTSGYNRSNMINPGSILETNTENLMRMVSYCENDVDCRRLLQLVHFGEKFNSSTCHKTCDNCLKITNFIEKDVTEIAKQLVELVKLTGQRFSSSHILEVYRGSFSQMVKKNRHETVSLHAAGKHLAKGEASRILHHLVVEDILVEEVKKSDFYGSISSILKVNEPKVCNLFAGHRIILRFPSSVKATKPGKSDATPAKGSLTSGKQNVFPIDTPQPQTEVDLNLSAKLYTALRMLRTTLVKEAGDSVFAYHIFGNATLQQISKRVPRTKEELLDINGIGKAKVSKYGDKILETIENTINEYYKLDKGSSGSKGSADSAKRRRDGDPDADADEEALTNSTGRSKKRTIKRQNRKAVIYDSADEDYFHGCHDEDLDFDLIEIDAIDQVTCKNGDGRVLPQWTTS

SEQ ID NO: 20 - protein, 1198 aa, Prunus persica
MSSMACRIQNIGRLPSAQVQKAWHALSNLQISHRNYTKPGKTVLVKDASSRYCRDVGRTATPSSCDIDKSHTHMQTHQYINGTNSRNSEAATCLGNRFPSSNVNVADVGNFFGGQSQVRASMVNNFDSRVPGGSFSNNSVHTSQIKHSAKVLVNDIDDDDEILENIDVDQIVEQYQSNCTPQPLISKLPPITPSIDKDSIARQEVTSLPPDLCSNCIHGLKIGLCPEAASHLQEMKDTLITISNELLDDVNDLSPTRIEKLRQDRLQLNKKIQQLERHLCNNSLDEERRKSHFSASTATPRPFQYETPQAAAFRTDTMIFDSQVQSHNVPGDYERCNSSSVSFSSVDGFGFSSCPVEREPYIPKFVEVNYIEGSNDNKWSSNNFPWTKKLEANNKKVFGNHSFRLNQREVINATMSGYDVFVLMPTGGGKSLTYQLPALICPGVTLVISPLVSLIQDQIMHLLQANIPAAYLSANMEWTEQQEIFRELNSEYCKYKLLYVTPEKVAKSDVLLRQLENLNARQLLARIVIDEAHCVSQWGHDFRPDYQALGILKQKFPNTPVLALTATATASVKEDVVQALGLVNCIVFRQSFNRPNLWYSVIPKTKKCLDDIDKFIKENHHDESGIIYCLSRMDCEKVAERLQECGHKAAFYHGSMDPAQRAFVQKQWSKDEINIICATVAFGMGINKPDVRFVIHHSLPKSIEGYHQECGRAGRDGQRSSCVLYYSYSDYIRVKHMISQGVIEQSPLASGYNRTNTANSGRVLETNTENLLRMVSYCENDVDCRRILQLIHLGEKFDCTTCKKTCDNCLKIKSFVEKDVTGIAKQLVELVKLTGQQFSSSHILEVYRGSFSQFVKKHRHQTVSLHGVGKHLAKGEASRVLRHLVTEDLLSEEVKKSDVYGSVSSILKRCMQYWGRFCSFFNTNIIIHFAADGTLDVFYVVFWLLGSSQVCHRPYDCDEHACLCRIIRFPSSVKASKQKNSEVISAKGSLTSGKQSPPHIGTEQPQSKANLDLSTKIFTSLKMLRTNLVRESDDGVMAYHIFANTTLQNMSSRIPRTKEELLEINGIGKGKLAKYGDRILETIEAAIKEYYKTDKNSTSSNDSNDMKRKRDGNNNGNENFDDNDFTKSTDRSKKKAPKRQNKTIEAYSYAEPDYPQLIDDELDLYCYDFEVNASDMKTNQNAGGRVLPQWSTPGNGRQ

SEQ ID NO: 21 - protein, 1233 aa, Ricinus communis
MTRENHMRQNLSISAEGFKCDEKLPKINWSQHDKAHDNFSCQKKFLSSNFLYSLENQKPHSEGVMAMRLTCQIQSFQRLQSPQVEKAWHALSCLQISCRNYLQPGKTGPLKNANLLQDVGQRPTFCSSSDGGKYSECLHVHQNFSESGAKNNKSERYMGNYVPQDNATAAETGNGLQRQSQIKASAANNTESKTFSGSFSDHSVYTSHNKESAEASTDFIDDDDLLGNIDVDQIVMEHNQSNCTPPNSKFPSITPTADKHNFARSDEMFLPTELCQNCNHGFKLGLCPEAGNHLQEMKDMLIAVSNELLDNSTNLSSVQIEKLRQDRLQLNKQIQQLESYLRDKERQKSHFSASTANQNFQYETPQCAANKIDPMRFDAQVYLRNESGGYESWNTPSISFSSVDRFGISSGPIEREPYIPKFVEVNYIEGSNDPKWSSTNFPWTTKLEAYNKKVFGNHSFRPNQREVINATMSGFDVFVLMPTGGGKSLTYQLPALVCPGITLVISPLVSLIQDQIMHLLQANISAAYLSANMEWAEQQEILRELSSDYCKYKLLYVTPEKVAKSDVLLRNLESLNARGLLARIVIDEAHCVSQWGHDFRPDYKELGILKKKFEKTPVLALTATATASVKEDVVQALGLVDCIIFRQSFNRPNLWYSVVPKTKKCLDDIDKFIKENHFDECGIIYCLSRMDCEKVAEKLQECGHKAAFYHGNMDAAQRAFVQKQWSKDEINIICATVAFGMGINKPDVRFVIHHSLPKSIEGYHQECGRAGRDGLRSSCVLYYSYSDYIRVKHMIVQGQIEQSPWTPGYNRINNTNSDRILEKNTENLLRMVSYCENDVDCRRILQLLHFGEKFNSGNCKKTCDNCSQIKALVEKDVTETAKQLVQLVKLTGQQFSSSHILEVYRGSLNQYVKKYRHETLSLHGAGKHLSKGEASRILRHLVTDDFLQEDVKKSDVYGSVSSILKVNESKAYNLCSGGQTIILRFPSTMKASKPSKFDATPAKGSLTSGKQSPPEVDSPAQAQPEVDLHLSAILYSALRMLRTLLVKEAGEGVMAYHIFGNATLQHLSKRIPRTKEELLEINGIGKAKVSKYGDRLLETIESTIKEYYKTDKNSSSSNGSNDSVKRRRDASRAPNGNAEEADDFTKSTGRSKKRVAKLQNKDTDIYTSRETNNSQCLDDDLDFEDSCHDFETNGSAIEAGKNDAGRVLPSWSTPGNKVKSSIPNLYQQYATKS

SEQ ID NO: 22 - protein, 1154 aa, Sorghum bicolor
MQANKSPRVNWPQHENAVQGFSSRDGFLSSSFLFSLPTQKPSPEAPESMLSLRSSACKIQGSERFHAPLIEKAWRSLCNTQAARKSYLRPGLSAKVKDCDRGHARTCGEGSYNTNKMATVSGNRMPSVESTSQPTERISLQNNSSHQPVGISSSMRSYQSNHVAQEDTRATNQYNFARTDAALHQSAPVADNMCTYDNYDAMDDDILASIDVDRIVMEHYQATPRGSSHNMSTPPGNKCSFNGMDEANLPRELSELCSHQCKLAFCREAMTHLQEMKDELLAVANELLDDDGELNPQHSQELHQRRLHLKKLVQLLEDHMTRSAQDEERQISHSMASTKATQQHLPPMTPGSTFITDSNRFQSQVYIGNGPRDSDLCYSSAPYSCSDNLSTPLNSVWKSYTPKVIDINYTEGSGDRKWSSTNFPWTKDLEAKNRNKFGNRSFRPNQREIINATMSGYDVFVLMPTGGGKSLTYQLPALISVGLTLVVCPLVSLIQDQIMHLSQANIPATYLSGNLDWSEQQEIMRDLKSCRYKLLYVTPEKIARSGALSGLLRDLDSQGHLSRIVIDEAHCVSQWGHDFRPDYKELGVLKQNFPKTPVLALTATATARVKEDVVQALALENCIVFKQSFNRPNLRYYLRPKTKKCVEDIDMFIRENHYKECGIIYCLSRMDCEKVSEKLRECGHTVAHYHGSMDPVNRTRIQEDWSKDKINIICATIAFGMGNLIFQTPVYVTSIIGCSILIGQTVGINKPDVRFVIHHSLPKSIEGYHQECGRAGRDGQPSSCLLYYQYSDYVSYCENDVDCRRLLQLIHFGERFDPSLCAKTCDNCLKESGWVEKDVTNIARQLVDLVTMTGHSNSSTHILEVYRGSVSQNVKKQRHDALPLHGAGKHLAKGEAARIMRHLVTEEILIEDVKKSDMFPAPGKASKMGNLDTSLFPQINKTVQQQSEVDEKLASILYEALLTLRRQIMEECSEGCHAYHIFKTDTLKEMSIRVPRTKEELLDINGIGKTKLKKYGDRVLATIEDFLSKHPNPRRNISGSGGKEHSEAAKKRRGSTASSAVSCGDDDFEEPTGQSKKRAAKTRTVSDAASMVHGARCIDADLDGPEVVDVDEHCSVPKPVASGRVLPKWAPAKAKSKGSSVPPSNLFHEFGYAK

SEQ ID NO: 23 - protein, 1166 aa, Setaria italica
MQANNNPPRVNWQHHANAIEGSSSKDDFLSSSFLFSLPTQRPNPEANREGMLSLRSSACKIQGTERLQVPWIEKAWRSLCNTQVACRSYLRPGLSAKVKDCDKGHARIYGEGSYNINKMETVPGNRILSQESTHRPCESGSVENNSIHQPTGIDSSTRTYQSNHVVQTDIMRARNQYNYVRTDAGLHQAAPVADSMCTDDKLDAMDDDDILASIDVDRIVMEHYQAMNTPRGSASQNTSTPPGNKCNFNGIDETNLPQELSELCNHQCKLAFCPKAMDHLQEMKNEMIAVADELLDDDGKLNLQRSEELRKKRLHLKKQIQLLEEYMARSSQDEERQRSHSMASTAAIQGHLPPMTPGSTFMMDSSRFQSQVYIRNGPGNSDLCYSPAPYSCSDNLSMPLHSVWREYTPKVIDTNYTEGSADKRWSSTNFPWTKELEAKNRNKFGNRSFRPNQREVINATMSGNDVFVLMPTGGGKSLTYQLPALISEGLTLVVCPLVSLIQDQIMHLSQANIPATYLSASMEWPEQQEILRGLMSCHYKLLYVTPEKIAKSNSLTGLLDNLYSQGHLSRIVIDEAHCVSQWGHDFRPDYKNLGVLKQNFPKTPVLALTATATARVKEDVVQALGLANCIVFRQSFNRPNLRYLLRPKTKKCLEDIDNFIRTNHFKECGIIYCLSRMDCEKVAEKLRECGHSVSHYHGSMDPVDRTRVQKQWSKDKINIICATVAFGMGNLIFQTSVCITSIVGCPMLMECGRAGRDGLPSSCLLYYQYSDYVSYCENDVDCRRLLQLIHFGEMFDPSRCAKTCDNCLKELTWVEKDVTNIARQMVELVTMTGQSHSSSHILEVYRGSVSQNVKKQRHDALPLHGAGKHLAKGDAARIMRHLVTEGILIEDVKKIDRHIFLSENDLLLVLFFLYLGIHLFLICYLLFNEKFPAPDKASKMGKLDASLFPQINKTVQQQSEVDENLSSMLFDALLSLREQIMDECNEGYHAYHIFKKDSLKEMSIRVPRTKEELLEINGIGKAKVKKYGDRVLATIEDFLSKHPNPRRNSSGSGSNEHTEAKKRRGFTASYAGSIADDDFEERTAQSKKRAAKTRSTKQGVSDATSMVHGARCMDADLDGVEVLDDELCSIQKPVASGRVLPKWAPAKAKGSSVPPSNLFQEFGYVK

SEQ ID NO: 24 - protein, 1180 aa, Solanum lycopersicum
MSKDKLPKANWTQHAIAHDNFSCQDKFLSSNILFSLPTQRHCARDEMNARSVTCHIRSVSKLEAEKAWKLLTSLKLSPKSYTRPGKTPQLTKDTNAFSQHSNHTQFPRASDGNCAPARCRPVHQGVGDDGENSDSRRYAGNCFPPHSSGVAETGNVVNRQSGVDNSHARGVGEISSSHANGASKKTREVYTTCADETEEDDILLNIDVDQIVEHYQTNCTPQPSVSRFPSTTPVTKSQSLAGHEETNLPPELSINCNHGLQLGLCPGALDHLQEMKDKLIEISNDLLDNVSDLSSEQIEMLRQERSQLKLQIQHLEKFLQTVSGNEERKMSQCSASTLTSAFQYETPSAFQYATPSSFPSRINPTRLDTQFSGYNESSHFDNWNSSSLSFDVTGGNGLSTAPVEREPYIPKYLEVNYIDGSNDKKWSCRDFPWTKKLEANNKKVFGNHSFRPNQREVINATMSGNDVFVLMPTGGGKSLTYQLPGLICPGITLVISPLVSLIQDQIMHLLQVNIPAAYLSSNMEWTEQQEILRELNSDGCKYKFLYVTPEKVAKSDVLLRHLESLHTRDTLARIVIDEAHCVSQWGHDFRPDYQCLGILKQKFPTVPVLALTATATISVKEDVVQALGLANCIIFRQSFNRPNLRYTVIPKTKKCLEDIGTFIKNNHFDQCGIIYCLSRMDCERVAEKLQEYGHKAAFYHGSMDGAQRANIQKQWSKDEINIICATIAFGMGINKPNVRFVIHHSLPKSIEGYHQECGRAGRDGLPSSCVLYYSYSDYIRVKHMISQGTVEQSPFGSGYGRSNVAASGRNLETNVENLLRMVSYCENEVDCRRLLQLIHFGEKFESTNCRKTCDNCCKTQNCIEKDVTEVAKQLVELVKTTGQKFSSAHVLEVFRGSLSQYVKKHRHESLHLHGAGKKLAKGEASRVLRHLVTEDILVEDVKKSDLYGSVSSVLKVNESKAYNLFAGGQTLRLRFPSFVKASKLGKYEATPAKGSLTSGKQSPPRTDPSGVPQSTFDPSLSAILYSALRKLRTNIVRESGDGVMAHHIFGDDTLQLIGQKVPRTKNELLDINGIGKVKINKYGDNVLQTIEATVRDYYKSDKTSSSGNDNTDSGKKRRNSINVQNGNSKDEEFFTESTGCTKKRVLKKQNKHAEVIDYRDLGYFDECIDGDLDFDETMMP

SEQ ID NO: 25 - protein, 1250 aa, Theobroma cacao
MSLFVLKLARTVYSRLLHGEVLEQWNFYQQFRIYVSQWPRKNIRVKAIQVKVTKMNDKLPKINWLSHVDAHDNFSCQKKFLSSNFLCSLETQKPCTEEEIRARLRVCQIQNSQKVQHPQVEKAWQILSSLPTSCRTYLRPGTTAPVKNSNDEISHNWRGRSTLTNSSDMKWSKHMHVSRNVNETDGKINEVGRCMASSFPSSNANAVEDGNHLQRHSEIKASMSNRSNSKVLGGSLWNHIVHASQLEQSAEVLADEIDDDDLLKDIDVDQIVSKHYQSTCTPQPSVSKFPPIAQMDKRAFAGEEEACLPTELCSNCSHGCKLGLCPEAASHVQEMKDKLIAVSNELLDNASNLSPEQIEKLREDRLQLNKQIQQLERYICDMERQKSHFSASTATRTFLYGTPQTASFSIDPIRFDAQVHLCNEPNGYENWNSSSVSFSSVNNFGVSSGPMEREPYVPKIIEVNYIEGSNDQKWSSRDFPWTKKLEANNKKVFGNHSFRPNQREVINATMSGCDVFVLMPTGGGKSLTYQLPALICPGITLVISPLVSLIQDQIMHLLQANIPAAYLSANMEWTEQQEILRELTSDYCKYKLLYVTPEKVAKSDVLLRHLDSLNARDLIARIVIDEAHCVSQWGHDFRPDYQGLGILKQKFPKTPVLALTATATASVKEDVVQALGLNNCIIFRQSFNRPNLWYSVIPKTKKCVDDIDKFIKENHFDECGIIYCLSRMDCEKVAEKLQECGHKAAFYHGNMDPAQRAAIQKQWSKDEINIICATVAFGMGINKPDVRFVIHHSLPKSIEGYHQECGRAGRDGQRSSCLLYYSYSDYIRVKHMISQGAAEQSPFVSGYSRFNNSGRILETNTENLLRMVSYCENDVDCRRLLQLLHFGEKFDSGNCKKTCDNCCRVKGFVDKDVTNIAKQLVELVKLTGQQFSSSHILEVYRGSLSQFVKKHRHETLSLHGAGKHVAKGEASRILRHLVIEEFLVEDVKKSDIYGSVSSVLKVNESKVQNLCVGGQTIILRFPSTVKATKLSKSEVTPAKGSLTSGKLSPPRVDTPAQSQSKVDLNLSAKLYSALRMLRTVLVKEAGDGVMAYHIFGNATLQHISKRVPRTEEELLEINGIGKAKISKYGDRILETIEVTIKEHYKTDRNSSSSNDSNDSTKRRRDANGAPKANVDDDDFTRSTSRSKKRTVKMQNNDGGAHSSKDPDYNNQCTGNDLDFDDYDDYGVESKCPEMKVHVDGTGRVLPSWST

SEQ ID NO: 26 - protein, 1235 aa, Vitis vinifera
MHIDQNDMIFISIKVHIAQNGMIFESIQMCSNIVANFFRPMICQIQHIQRLQSLQVEKAWGALSSLKLSSRNYSKPGKMAPLLKDASVEFPRDVRKCNLQSSHNTNNQYLEHNLPHQNLGETNSSYSETASCRGNSFRSGSACAENAGREGGQNETKPSMLYNSHIQVVGQSSGTCNVHTGQVKELVGAFPNGTDDDDILEDIDVDQIVMEHYQSTCTPQPSISKLPPVTPTLSTVNIAKHEETFLPLELCSNCSHGFKLGLCPEAANHLQELKDMLIVISNELLDNVDLTSVQVEKLRQDRLYLNKQIQQLEIHLHSVSVDEERKNSNFSASTTTPWAQFQTPPATAVGIDPMRFDAQVHLRNEPGNYEKWNTSSVSFSSIDRFGVTPYPLEREPYIPKLIEVNYIEGSSDKKWSSGNFPWTKKLEANNKKVFGNHSFRPNQREVINATMSGYDVFVLMPTGGGKSLTYQLPALISPGITLVISPLVSLIQDQIMHLLQANIPAAYLSASMEWNEQQEILRELSSCKYKLLYATPEKVAKSDVLMRNLDNLHARELLSRIVIDEAHCVSQWGHDFRPDYQGLGILKQKFPNTPVLALTATATASVKEDVVQALGLVNCIIFRQSFNRPNLWYSVLPKTRKCLDDIDKFIRENHFDECGIIYCLSRLDCEKVAERLQECGHKAAFYHGSMDPARRAFVQKQWSKDEINIICATVAFGMGINKPDVRFVIHHSLPKSIEGYHQECGRAGRDGQRSSCVLYYSYSDYIRVKHMITQGVVEQSPLASGQNRSNMASSGRILETNTENLLRMVSYCENDVDCRRLLQLVHFGEKFDSAHCKKTCDNCLKIKSFVEKDVTEIAKQLVELVKLTREQFSSSHILEVYRGSLSQYVKKHRHETLGLHAAGKHLAKGEASRILRHLVTEDFLMEDVKKSDIYGSVSSVLKVNESKVYKLFSGGQKIILRFPSSAKSSKLSNFEATPAKGSLTSGKLSPPRIETPAHLPEVDLNLSAKLYSALRILRTVLVKEAGEGVMAYHIFGNATLQQISKRIPRTKEELLEVNGIGKAKISKYGDRVLETIESTIKEYYKTDKNSSSSNDSTDTIKRRRESAKVLDANPEDDDFTKSTDRSRGRAMKRHNKGGEANNTRETDYYNQCIDDDLDFDDANCDVAINGSAPKVDRDGARRTLPSWSTPSNKGHDQHLNMFQEYSFKGTHIKAGKMKDVGQFAVAIEFVLVFLL

SEQ ID NO: 27 - protein, 923 aa, Arabidopsis lyrata
MSRRGGGPVTVLNVAEKPSVAKSVAGILSRGTFRTREGRSRYNKIFEFDYAINGQPCRMLMTSVIGHLMELEFANRYRKWHSCDPADLYQAPVMKHVPEDKKDIKKTLEEEARKSDWLVLWLDCDREGENIAFEVVDVCRAVKHNLFIRRAHFSALIDRDIHEAVQNLRDPNQLFAEAVDARQEIDLRIGASFTRFQTMLLRDRFAIDSTGEERSRVISYGPCQFPTLGFIVERYWEIQAHEPEEFWTINCSHQSEEGLATFNWMRGHLFDYASAVILYEMCVEEPTATVMNVPHPRERFKYPPYPLNTIELEKRASRYFRLSSEHTMKVAEELYQAGFISYPRTETDSFSSRTDLCAMVEEQRRHPAWGSYAQRLLEPEGGLWRNPGNGGHDDKAHPPIHPTKFSSGESNWSRDHLNVYELVVRHYLACVSQPAKAAETTVEIDIAGERFSASGRAILAKNYLEVYRFESWGGSVIPVYEKGQQFIPTTLTLDSAVTRPPPLLCEADLLSCMDKAGIGTDATMHDHIKKLLDRGYATKDANTRFSPTNLGEALVMGYDDMGYELWKPNLRALMERDMNEVSVGRKTKAEVLETCLQQMKACFLDARVKKSKLLEAMTIFFERSNNTDESESQTAGEVIRRCNLCNESDMALRKNRDGNFMVGCMNYPQCRNAVWLPGPTLEASVTTDVCQTCGPGPVYKILFKFRQIGIPPGFDVNHLGCIGGCDDILKQLIDICGTGSRSQARRAPGTVPSNNIQGSNTRQGNFCIHCQQRGHASANCPSRATAFRNSRLTATNPRNDESTVSCNTCGTQCVLRTANTEANRGRQFFSCPTQGCSFFAWEDSINNSSGNATTGSNSGGSGRRGRGRGGRGGQSGGGRRNSGTSFVSATGEPVSGIRCFSCGDPSHFANVCPNRNNSNGNYY

SEQ ID NO: 28 - protein, 924 aa, Brachypodium distachyon
MHPSGGGGGAIRVLNVAEKPSVAKSVAEILSRRAMQSRPGRSRYNRIFEFNYAIGGQACHMLVTSVTGHLMELDFDDRYRRWYSCDPVELFHAPVRKAVPQDKLDIKRTLEEEARTCQWLVLWLDCDREGENIAYEVVEICAGVNHCLNIWRARFSALIDREIHEAVQHLGRPNKLFADAVDARQEIDLRIGASFTRFQTMLLKDAFVLDVSGEERNMVLSYGPCQFPTLGFIVERFWEIQAHEPEEFWTINCSHTSDEGTASFGWIRGHLFDYSSAIVIYEMCVQEPMATVQNVRNQEKLKYPPYPLSTLELQKRASRCCRMSSEHTMKVAEELYQAGFISYPRTETDNFSPNTDLHAIAHEQVPHPVWGSYAQRLLNPEERLWRNPSNGGHDDKAHPPIHPTKFTAGESNWSQDHHKVYELVVRHFLACCSQPAVGAETTVEIDIAGEQFNASGRVVLAKNYLDVYRYDSWGGSLLPTYTIGQQFVPTTLTLDSGVTRPPPLLAEADLLSCMDKAGIGTDATMHEHIKKLLDRCYATKDANSRFSPTNLGEALVMGYDEMGYELWKPYLRAMMEADMKAVSIGTKSKLEVLEGCLQQMKACFLDARSNKVKLLDAMGTFFARSNRPLNETQNPMEVVRPCGACNDSEMLLKRKPNGGFMVGCRSFPQCRNVVWLPGSLSEAAVTEQICPTCVPGPVYKIQFKFNRRDIPPNFDVDHLGCIGGCDDVLKELIEITRFVNHNQTTTPARGQSQTPSGVRQGAPRQDLHPGFRPAGQFANGHTPVVNPQGFRSTHTQNSRNASGQVLCTTCGEACISRTANTEANRGRKFYKCQDSGCGFFAWEDELENVVPRGRGRGGRGGGRQASASAGRRGGTQGRGRRGRGRNADANGMTFVSATGDTVHGCCFACGDPSHFANACPNRGR

SEQ ID NO: 29 - protein, 915 aa, Fragaria vesca
MLTEFGAELGWGWLSVDGGWLPKAEAVVWNKQAAVEDWACLCWREMVRVLNVAEKPSVAKSVANILSRGQGLRMREGRSRYNKIYEFNYSINGCHCQMLFTSVTGHLMELEFEDRFRKWHSCDPALLFQAPVRKFVPEDKLDIKRTLEEEARNCQWLVLWLDCDREGENIAFEVIDVCTSVNRHLTIKRARFSALIDRDIHHAVQNLDNANKYFADAVDARQEIDLRIGASFTRFQTMLLRDAFVIDSATDDRNLVLSYGPCQFPTLGFIVERYWEIQSHEPEEFWTINCSHRSDEGTATFGWMRGHLFDHACAVIIYEMCVEDPIATVTKVRQQEKPKYPPYPLNTIELEKRASRYFRMSSEHTMKVGTVGVAEELYQAGFISYPRTETDGFSPRTDLHAIVQEQQGHPGWGSYAQRLLDPASGLWRNPSSGGHDDKAHPPIHPTKFSAGESNWSQDHNRLYELVVRHFLACVSQPAVGAETTVEIDIAGEMFSASGRVILAKNYLDVYRFESWGGSLLPTYAVGQQFMPTTLTLDSGVTRPPPLLSEADLLGCMDKEGIGTDATMHDHIKKLLDRFYATKDANTRFSPTNLGEALVMGYDDMGAVMERDMKAVSEGNKSKAEVLETCLQQMKGCFLDARQNKVKLFEAMAVFFERSNRPGGDDQHTSGEFIRRCGLCQEADMVLRKNRDGNFMVGCMGYPQCRNAIWLPGSVSEAVATTNICNSCTPGEDNQLECASPSFVGIGLDSSSSSRCIGGCDEILRQLTEICGTGSRSAARGRGPTTSSNVQQNNTRQGACIYCHQSGHSSGDCPSQSSGPRSVRPRTMNAQSGMTAQLIWEDNVSNGNGGRGFQRANVSAGRGAGGRGSGGRGAQGAGHATGGTFVSATGDPNSGRRCFVCGDPSHFANVCPNRGN

SEQ ID NO: 30 - protein, 814 aa, Oryza sativa
MHHGGGGGAIRVLNVAEKPSVAKSVAEILSRPSGGMRSREGRSRYNRVFEFDYSIGGRACHMLVTSVTGHLMELEFDDRFRRWHSCDPADLFHAPVRKSVPQDKQDIKRTLEEEARKCQWLVLWLDCDREGENIAYEVIDICAGANSRLNIWRARFSALIDREIHEAVQHLDRPNKLFADAVDARQEIDLRIGASFTRFQTMLLKDAFVLDDTGDDRNIILSYGPCQFPTLGFIVERFWEIQAHEPEEFWTINCSHTSDEGTASFGWIRGHLFDYSSAVVIYEMCVEEPMATVQNVRNQEKLKYPPYPLSTIELQKRASRYFRMSSEHTMKVAEELYQAGFISYPRTETDNFSPNTDLHSIVHEQVAHPNWGTYAQRLLDPEARLWRNPSNGGHDDKAHPPIHPTKFSAGETNWTDNHKKLYELVVRHFLACCSQPAVGAETTVEIDIAGEQFNASGRVVLAKNYLDVYRFDSWGGTLLPTYIIGQQAGIGTDATMHDHIKKLLDRCYATKDANTRFSPTNLGEALVMGYDEMGYELWKPYLRSMMEADMKSVSIGTKSKSEVLENCLQQMKACFLDARANKVKLFDAMGTFFARSSRPVNETQNSIETVRPCAACNESEMFLKQRPCRNVVWLPRSLSGAAVTDQVCPTCAPGPVYKIQFKFRRRDIPPNFDVDHLGCIGGCDDILKELMELSRFGSHSQTATPARNQSQTASGVRQGSSRQDLHTSFHPAVQFTNGQTPVVNPQGFRSTHTQSSGNASDGKTMWRTLRRGAVAGVGGAGAVAAGNHLHLHLQGGEAAPKGEAGGAEDGMLMA

SEQ ID NO: 31 - protein, 910 aa, Populus trichocarpa
MIKVLNVAEKPSVAKSVATILSRNQLRVRDGRSRYNKIFEFNYSINGQQCHMLVTSVTGHLMEVEFEDRFRKWHSCDPADLYTAPVRKYVPEDKLDIKRTLEEEARRCHWLVLWLDCDREGENIAFEVMEVCKGVNRNLTIRRARFSALIERDIHEAAQNLIAPNQWFSDAVDARQEIDLRIGASFTRFQTMLLRDRFVIDSAQDDRNLVLSYGPCQFPTLGFVVERYWEIQSHEPEEFWTINCTHRSDEGLASFNWMRGHLFDYTSSVILYEMCVEEPTATVSNRNHQQEKLKYPPYPLSTIELEKRASRYFRMSSEQTMKVAEDLYQAGFISYPRTETDSFSSRTDLHTIVQEHQEHPVWGSYAQRLLDPGAGLWRNPSNGGHDDKAHPPIHPTKFSAGESRWSQDHHRLYELVVRHFLACVSQPAVGAETVVEIDIAGERFSASGRVILAKNYLDVYRFESWGDSMIPTYLQGQQFIPATLTLDSGVTRPPPLLSEADLLSCMDKAGIGTDATMHDHIKKLLDRFYVTKDANTRFSPTNLGEALVMGYDDMGYELWKPNLRSLMECDMKEVSVGNKSKAEVLATCLQQMKACFLDAKVNKVKLLEAMAIFFNRSDRSNGDDSSALGENVRPCGLCQEANMVLKKNRDGNFMVGCSGFPQCRNAVWLPGPVLEATITNNICNSCTPGPVYLIQFKFRQLEIPPGFNVNHLGCIGGCDETLRQLIEICGTGSRVQGGNGPPTTTPSNPQRSNSRQAPCIYCYQTGHASTDCPSRISATRHVQSHGMNQQNGESSIPCSTCGTPCVLRTANTANNRGRKFYSCSSQACNFFVWEDNLNNGSAPRSAPRPNMSNSASNPSRRGGRGRGVQNAGRAADVTFVSATGEPISGRRCFVCGDPSHFANACPSRGS

SEQ ID NO: 32 - protein, 833 aa, Ricinus communis
MINVLNVAEKPSVAKSVATILSRNQQHGLRVREGQSRYNKIFEFNYVINGQNCHMLVTSVTGHLMELEFDDRFRKWHSCDPADLYHAPVRKFVPEDKTNIKRTLEEEARRCQWLILWLDCDREGENIAFEVVDVCRSANRYLTVRRARFSALIDREIHEAAQNLVSPNQWFSDAVDARQEIDLRIGASFTRFQTLLLRDKFVIDSAQDDRNLVLSYGPCQFPTLGFIVERYWEIQSHESEEFWTINCSHTSVEGIANFSWMRGHLFDYTSAVILYELCVLEPTATVTKVQQKEKQKYPPYPLSTIELEKRASRYFHMSSEQTMKVAEDLYQSGFISYPRTETDGFSSRTDLHTIVRDQQAHPIWGSYAQRLLDPGTGLWRNPSTGGHDDKAHPPIHPTKFSPGETGWSQDHHRVYELVVRHFLACVSQPAVGAETTVEIDIAGEQFSASGRVILAKNYLDVYRFESWGGSMIPTYVHGQQFMPTTLTLDSGVTRPPPLLSESDLLSCMDKAGIGTDATMHDHIKKLLDRFYATKDANTRFSPTNLGEALVMGYDDMGYELWKPNLRSMMEYDMKEVSMGHKSKAEVLETCLQQMKTCFLDARINKVKLLEAMAVFFERSDRSSGNDNHATVDIVRQCGLCRETNMVLRRNRDGNFMVGCMGYPQCRNAIWLPGPIIEATVTTSVCNYCTPGPVYLIQFKFRQLEIPPGFSVNHLGCIGGCDDTLRQLTDICGTGSRVQARARAPNTTPSNSQQSNTRFATCVHCHQTGHASIDCPLQLSGSRRVQSRGTNEQMGESSVTCGTCGTPCALRTANTANNRGRKFYSCPSQSCNFF

SEQ ID NO: 33 - protein, 860 aa, Sorghum bicolor
MQPGGGGAIRVLNVAEKPSVAKAVAEILSRRSMQSRAGRSQYNRIFEFNYAINGRACHMLVTSVTGHLMELEFDERFRRWHSCDPAELFHAPVRKSVPQDKQAIKQTLEEEARRCQWLVLWLDCDREGENIAYEVIDVCTGANSHLNIWRARFSALIDREIHESVQHLGRPNKLFADAVDARQEIDLRIGASFTRFQTMLLKDAFVINVTGDDRNLVLSYGPCQFPTLGFIVERFWEIQAHEPEEFWTINCTHTSDEGTASFGWIRGHLFDYSCAISIYEMCVSEPMATVQNVRNQEKLKYPPYPLSTVELQKRASRYFRMSSEHTMKVAEELYQAGFISYPRTETDNFSPNTDLHAIVREQVNHPVWGAYAQRLLNPEARLWRNPSNGGHDDKAHPPIHPTKFSEGERNWSPDHIRLYELVVRHFLACCSQPAVGAETTVEIDIAGEQFNASGRVILAKNYLDVYRFDSWGGTLLPTYNIGQQFVPTTLTLDSGVTRPPPLLAEADLLSCMDKAGIGTDATMHDHIKKLLDRCYATKDENTRFSPTNLGEALVMGYDEMGYELWKPYLRSMMEADMKSVSMGTKSKSEVLESCLQQMKACFLDARVNKAKLLDAMGTFFARSNRPINETQNPVEVVRPCGACNGSEMVLKRRVTGEFMVGCRSYPQCRNVVWLPGSLSEAAVTNQVCPICAPGPVYKIQFKFRRRDIPPNFDVDHLGCVGGCDDILKELMELSRFGSRSQAATPGQVLCTSCGAACISLTANTEANRGRKFYKCQDPGCGFFKWEDELDNGTGRGRRGRGSSRQATASASAGRRGGGRRGRGRNADGGMFVSATGDTVPGCCFTCGDPSHFANACPNRR

SEQ ID NO: 34 - protein, 915 aa, Zea mays
MQPDGGGAIRVLNVAEKPSVAKAVAEILSRRSAQSRAGRSQYNRIFEFNYAINGRACHMLVTSVTGHLMELEFDDRFRRWHSCDPAELFHAPVRKSVPQDKQAIKQTLEEEARRCQWLVLWLDCDREGENIAYEVIDVCTRANSHLNIWRARFSALIDREIHESVQHLGRPNKLFADAVDARQEIDLRIGASFTRFQTMLLKDAFVIDVTGDERSLVLSYGPCQFPTLGFIVERFWEIQAHEPEEFWTINCTHTSDEGTASFGWIRGHLFDYSCAISIYEMCVSEPMATVQNVRNQEKLKYPPYPLSTVELQKRASRYFRMSSEHTMKVAEELYQAGFISYPRTETDNFSPNTDLHAIVREQVNHPVWGAYAQRLLNPEARLWRNPSNGGHDDKAHPPIHPTKFSEGERNWSPDHTRLYEFVVRHFLACCSQPAVGAETTVEIDIAGEQFNASGRVILAKNYLDVYRFDSWGGTLLPTYNIGQQFVPTTLTLDSGVTRPPPLLAEADLLSCMDKAGIGTDATMHDHIKKLLDRCYATKDENTRFSPTNLGEALVMGYDEMGYELWKPYLRSMMEADMKSVSVGTKSKSEVLESCLQQMKACFLDARVKKAKLLDAMGTFFARSNRPINETQNPVEVVRPCGACNGSEMLLKRRASGEFMVGCRSYPQCRNVVWLPGSLSEAAVTNQVCPICAPGPVYKIQFKFRRRDIPPNFDVDHLGCVGGCDDILKDLMEISRFGSRSQAATPARGPTPNGVGQGTPRQDLHTIFRPASQLNNDNPSVMHSQGFRSTHTQNPSNASDAGQVLCTSCGALCISRIANTEANRGRRFYKCQDPGCGFFKWEDEVDNGTGRGRRGRGSSRQASASASAGRRGGGRRGRGRNADGGMFVSATGDTVLGCCFNCGDPSHFANACPNRR

SEQ ID NO: 35 - protein, 930 aa, Thellungiella halophila
MSRRGGGPVTVLNVAEKPSVAKSVAGILSRGSFRTREGRSRYNKIFEFDYAINGQPCRMLMTSVIGHLMELEFSDRFRKWHSCDPADLYQAPVMKHVPEDKKDIKKTLEEEARKSDWLVLWLDCDREGENIAFEVVDVCRAVKQNLFIRRAHFSALIDREIHEAAQNLREPNQLFAQAVDARQEIDLRIGASFTRFQTMLLKDRFSIDSTGGEERSRVISYGPCQFPTLGFIVERYWEIQAHEPEEFWTINCSHESEEGLATFNWMRGHLFDYVSAVILYEMCVLEPTATVMNVPHPREKFKYPPYPLNTIELEKRASRYFRLSSEHTMKVAEELYQAGFISYPRTETDSFSSRTDLRAMVEEQTRHPAWGPYAQRLLEPEGGHWRNPGNGGHDDKAHPPIHPTKFSSGESNWSRDHLNVYELVVRHYLACVSQPAIAAETTVEIDIAGERFSASGRAILAKNYLEVYRFESWGGSVIPVYEKGQQFIPTRLTLDSAVTRPPPLLSEADLLSCMDKAGIGTDATMHDHIKKLLDRGYATKDANTRFSPTNLGEALVMGYDDMGYELWKPNLRAIMEHDMNEVSVGSKTKAEVLQTCLQQMKACFLDARVKKAKLLETMTIFFERSNNTDEGENQTAGEVVRRCNLCHESDMALRKNRDGNFMVGCMSYPQCRNAVWLPGPTLEASVTADVCQSCGPAPVYKIRFKFRQIGIPPGFDTNHLGCVGGCDDILKQLIDICGTGSRSQARTAPGASSNNFQGGNIRQNNTCIHCQQRGHTSANCPSRISGSRNPRPTTGTNPGNDETTVSCNTCGTPCALRTANTEANRGRRFFSCPSQGCNFFAWEDSISNGSGNATAGSNSGGSGRRGRARGRGNRGGQSGGARGGGGGRGGGGTSFVSATGEPVSGRRCFSCGDPSHFANACPNRNSNGNF

SEQ ID NO: 36 - protein, 919 aa, Capsella rubella
MSRRGGGPVTVLNVAEKPSVAKSVAGILSRGSFRTREGRSRYNKIFEFDYAINGQPCRMLMTSVIGHLMELEFSDRYRKWHSCDPADLYQAPVMKHVPEDKRDIKKTLEEEARKSDWLVLWLDCDREGENIAFEVVDVCRAVKHNLFIRRAHFSALIDREIHEAVQNLRDPNQLFAEAVDARQEIDLRIGASFTRFQTMLLRDRFAIDSTGEERSRVISYGPCQFPTLGFIVERYWEIQAHEPEEFWTINCSHQSEEGIATFNWMRGHLFDYASAVILYEMCVEEPTATVMNVPHPRERFKYPPYPLNTIELEKRASRYFRLSSEHTMKVAEELYQAGFISYPRTETDAFSSRTDLRAMVEEQTRHPEWGAYAQRLLEPEGGLWRNPGNGGHDDKAHPPIHPTKFSSGESNWSRDHLNVYELVVRHYLACVSQPAVAAETTVEIDISGERFSASGRAILAKNYLEVYRFESWGGSVIPVYEKGQQFIPTSLTLDSAVTRPPPLLCEADLLSCMDKAGIGTDATMHDHIKKLLDRGYATKDANTRFSPTNLGEALVMGYDDMGYELWKPNLRAIMEHDMNEVSVGRKTKAEVLETCLQQMKACFLDARVKKSKLLEAMTIFFERSNNTDEGENQTAGEVVRRCNLCNESDMALRKNRDGNFMVGCMNYPQCRNAVWLPGPTLEASVTTNVCQSCGPGPVYKILFKFRQIGIPPGFEVNHLGCVGGCDGILKQLIDICGTGSRSQARRAPDTVPPNNIRGSNTRQSNVCIHCQQRGHASSNCPSRVSASRNSRPTGTNPRNDESTVSCNTCGTQCVLRTANTEANRGRQFFSCPTQGCSFFAWEDGISNSSGNATTGSNSGGSGRRGNRGRGRGGRGGQSGGRRGSGTSFVSATGEPVSGIRCFSCGDPSHFANACPNRNS

SEQ ID NO: 37 - protein, 921 aa, Brassica rapa
MSRRGGGPVTVLNVAEKPSVAKSVAGILSRGSFRTREGRSRYNKIFEFDYAINGQPCRMMMTSVIGHLMELEFADRFRKWHSCDPADLYQAPVMKHVPEDKKDIKKTLEEEARRSDWLVLWLDCDREGENIAFEVVDVCRAVKQNLYIRRAHFSALIDREIHEAVQNLREPNQLFAQAVDARQEIDLRIGASFTRFQTMLLKDRFVIDSTGDEERSRVISYGPCQFPTLGFIVERYWEIQAHEPEEFWTINCSHESEEGLATFNWMRGHLFDYASAAILYEMCVLEPTATVMNVPHPREKFKYPPYPLNTIELEKRASRYFRLSSEHTMKVAEELYQAGFISYPRTETDSFSSRTDLRAMVEEQTRHPAWGPYAQRLLEPEGGLWRNPGNGGHDDKAHPPIHPTKFSSGESNWSRDHLNVYELVVRHYLACVSQPAVAAETTVEIDIAGERFSASGRAILAKNYLEVYRFESWGGSMIPVYEKGQQFIPTRLTLDSAVTRPPPLLCEADLLSCMDKAGIGTDATMHDHIKKLLDRGYATKDANTRFSPTNLGEALVMGYDDMGYELWKPNLRAIMEHDMNEVSVGNKTKAEVLETCLQQMKACFLDARVKKTKLLEAMTIFFERSNNSDEGENQTAGEVVRRCNLCHESDMALRKNQDGNFMVGCMSYPQCRNAVWLPGPTLEASVTTDTCQSCGPGPVYKIRFKFRQIRIPPGFDVNHLGCVGGCDDVLKQLIDICGTGSRSQARAAPGATPNNVRGSNIRQNNVCIHCQQGGHTSANCPTRASGYRNPRATGTANPRNNETTVSCTTCGTPCAIRTANTEANRGRKFYSCPSQGCNFFTWEDSISNGTGNATTGSNSGGSGRRGRGGGRGNRGGGQRGGGRGGGGTSFVSATGEPVSGRRCFSCGDPSHFANACPNRNS

SEQ ID NO: 38 - protein, 909 aa, Gossypium raimondii
MSGTIKVLNVAEKPSVAKSVSGFLSRNQALRVRDGRSRYNRIFEFNYSIRGQPCHMLFTSVTGHLMELEFEDRFRKWHSCDPLDLYHAPVRKFVPEDKLDIKRTLEEEARRCQWLVLWLDCDREGENIAFEVINVCRAVNRHLTIRRARFSALIDREIHHAMQNLIDPNPWFSDAVDARQEIDLRIGASFTRFQTMLLRDKFVIDSATDDRNLVLSYGPCQFPTLGFVVERYWEVQSHEPEEFWTINCSHRSDEGVATFNWMRGHLFDYTCAVIVYEMCVQEPTATVTKVQHKEKLKYPPYPLNTIELEKRASRYFRMSSEHTMKVAEELYQAGFISYPRTETDCFSSRTDLHAIVQEQQGHPDWGSYAQRLLDPETGLWRNPGSGGHDDKAHPPIHPTKFSTGEHGWSQDHRTLYELVVRHFLACVSQPAVGAETTVEIDIAGELFSASGRVILERNYLDVYRYESWGGSMIPTYTVGQQFVPASLTLDTGVTRPPPLLSEADLLSCMDKAGIGTDATMHDHIKKLLDRFYATKDSNTRFSPTNLGEALVMGYDDMGYELWKPNLRSMMEFDMKEVSVGNKSKDEVLATCLQQMKACFFDARLNKVKLLEAMAVFFERSNRAVGGDNYAAGEVVRQCDLCQESSMVLKKNRDGNFMVGCSGFPQCRNAIWLPGSILEAAVTSNICSSCNPGPVYLIQFKFRQIEIPPGFNANHLGCIGGCDDTLRQLIEICGTGSRMSARGRGPTTTSSNGQRSSNRHNSCIHCQQTGHSSNDCPSQFSRSRNSQSHTNSENGDPSVSCSTCGMPCVLRTANTANNRGRKFYSCPSQECNFFIWEDGVSNGNGGRSIPSTNCSASNSGRRGGRGQSGRNRSHAADTTFVSATGDPVSNRCYVCGDPSHFANVCPNRGM

SEQ ID NO: 39 - protein, 914 aa, Theobroma cacao
MSGTIKVLNVAEKPSVAKSVSGILSRNQGLRVRDGRSRFNRIFEFNYSVRGQPCHMLFTSVTGHLMELEFEDRFRKWHSCDPADLYHAPVRKHVPEDKMDIKRTLEEEARRCQWLVLWLDCDREGENIAFEVIDVCRAVNCHLTIRRARFSALIEREIHHATQNLVDPNPWFSDAVDARQEIDLRIGASFTRFQTMMLRDKFVIDSATDDRNLVLSYGPCQFPTLGFVVERYWEVQSHEPEEFWTINCSHKLDEGVATFNWMRGHLFDHTCAVIVYEMCVQEPNATVTKVRHQEKLKYPPYPLSTIELEKRASRYFRMSSEHTMKVAEDLYQAGFISYPRTETDCFSSRTDLHAIVQEQQDHPEWGSYAQRLLDPGTSLWRNPSSGGHDDKAHPPIHPTKFSAGEHNWSQDHRKLYELVVRHFLACVSQPAVGAETTVEIDIADEQFSTSGRVILERNYLDVYRYESWGGSMIPTYTLGQQFIPTSLTLDTGVTRPPPLLSEADLLSCMDKAGIGTDATMHDHIKKLLDRFYATKDSNTRFSPTKLGEALVMGYDDMGYELWKPNLRSMMEFDMKEVSVGNKRKDEVLATCLQQMKACFLDARLNKVKLLEAMAVFFERSNQSAGDDNHVAGEVVRQCGLCRESSMVLKKNRDGNFMVGCLGFPQCRNAIWLPGSVLEAAVTSNICGSCNPGPVYLIQFKFRQLEIPPGFNANHLGCIGGCDDILRQLIEICGTGSRMSARGRGPTTTSSNVQRNSSRQGACLYCQQTGHSSNDCPSQFSGSRNSRSRTSSQNGEPSVSCSTCGTPCVLRTANTANNRGRKFYSCPSQECNFFIWEDEHNNGTGGRSIPRAGINGSASNSSRGGGRGRGRFGQNGARAADVTFVSATGDPISGRRCYVCGDPSHFANVCPNRGM

SEQ ID NO: 40 - protein, 915 aa, Eucalyptus grandis
MSGGGRAINVLNVAEKPSVAKSVATLLSRGQGMRVREGRSRYNKIFEFDYGIRGQRCRMLVTSVTGHLMELEFEDRFRKWHSCDPADLYAAPVRKSVPQDKLDIKRTLEEEARRCQWLVLWLDCDREGENIAFEVIDTCTAANCNLTIKRARFSALIEREIHDSVQNLVEPNRWFADAVDARQEIDLRIGASFTRFQTMLLRDAFVIDSAADDRNLVLSYGPCQFPTLGFVVERFWEIQSHEPEEFWIINCSHKSEEGIATFNWTRGHLFDYTCAVIIYEMCVEEPPATVAGVRQQEKYKYPPHPLSTIELEKRASRYFRMSSEHTMKVAEELYQAGFISYPRTETDNFSARTDLHAIVQEQRGHPVWGSYAQRLLDPSSGLWRNPSNGGHDDKAHPPIHPTKFSGGERNWSQDHHRLYELVVRHFLACVSQPAVGAETTVEIDIAGEQFAASGRVIIAKNYLDVYRFESWGGSVIPTYVPGQQFIPTTLTLDSGVTRPPPLLSEADLLNCMDKAGIGTDATMHDHIKKLLDRFYATKDQNMRFSPTNLGEALVMGYDDMGYKLWKPNLRSMMEFDMRAVSEGAKTKAEVLETCLQQMKACFLDARSNKQKLMEAMAVFFERAARTARDEQHVVGEFVRLCGLCHQSNMVLKRNRDGNFMVGCLGFPQCRNVVWLPGSVSEAVVTANICNSCSPGPIYMIQFKFRRLEIPPIFSVDHLGCIGGCDDTLQQLTEICGTGSRMSAARGGGPTPLSSSAQRSNSRQQACSSCRQLGHSSTDCPSVISGTRNSRSRRADQQDGGLSVSCDTCGASCPMRTANTANNKGRKFYSCQSEGCNFFVWEDSLQNGGGRHGANGGASNSRARSNSLGGRGRGGRGGNNATNGTFVSATGDPVTGRCYVCGDPSHFANACPNRFT

SEQ ID NO: 41 - protein, 913 aa, Glycine max
MNVLNVAEKPMVARTVATILSRNQNMRMREGRSRYNKIFEFNYTIRGQPCHMIFTSVTGHLMELEFDDRYRKWHSCDPADLFRAPVHKFVPEDKKDIKRTLEEEARRCQWLILWLDCDVEGENIAYEVIDVCTAVNPHLTIKRAWFSTLIDRDIHNAAQNDLRDPDKRVADAVDVRQEIDLRIGASFTRFQTMLMKDAFIIDTATDDRNRVLSYGPCQFPTLGFVVERFWEIQAHEPEEFWSIICSHESKEGTAEFSWMRGRLFDYTCAVIIYEMCVEEPTATVTNIRQQEKPKYPPFPLNTIELQKRASRYFRMSSDHTMKVAEELYQAGFISYPRTETDSFSPGTDLHTIVQEQQGHPEWGIYAQRLMDPEAGLWRNPRGGGHDDKAHPPIYPTKFSTGESGWSQDHRKLYELVVRHFLACVSKPALGAETTVEINIAGELFSACGRVILEKNYLDVYRYESWGGSMIPTYTNGQQFNPTKLTLESGVTRPPPLLSEADLLSYMDREEAKIGTDATMQDHIKKMLDRSYATKDSSTRFTPTNLGEALVLGYDDIDMTYKLWKPDLRSEMEKKMDDVKKGDKSKAEVLVTILQKMEACFLEARLNKVKLLEAMAIFFERSTRSSSDELHATGEVVRRCGLCQESDMLLRKNRDGNFMVGCMGYPQCRNAVWLPGSVSEAVVTTNTCNFCTPGPVYLIQFKFRRLEIPPNYSPNHLGCIGGCDEILAQLTEICGRGPRMPARPRGPTAPTSNAHHTNPRQGACMNCRETGHSSTDCPLRYGNVQHHGTSEHNGEASVSCSSCGTPCVLRTANTVNNRGRKFYSCQSQECNFFVWEDSLNAGTGGRSVTRSNSIPALNPRQTGGRGSRGRGGQYGSRTANTTFMSATGDPISGRRCYTCGDPSHFANVCPHRGV

SEQ ID NO: 42 - protein, 923 aa, Mimulus guttatus
MAGGGGRPLRALNVAEKPSVAKAVSGILSKNPSSGGLRVREGRSRYNKIFEFNYAIQNQQFQMSFTSVTGHLMELEFEDRYRKWHSCDPVDLYHAPVRKHVPQDKSDIEKTLEEEARKCQWLILWLDCDREGENIAFEVVEACLRTNRNLNIWRARFSALIDREIHDAVQHLVRPNQLFADAVDVRQEIDLRIGASFTRFQTMLLKDAFVLDFATEERNVILSYGPCQFPTLGFVVERFWEIQSHEPEEFWTINCTHNSEEGTATFSWMRGHLFDYTCATIIYEMCVLEPNATVTNVRNQEKPRYPPHPLSTIELEKRASRYFRMSSEQTMKVAEDLYQAGFISYPRTETDSFSVRTDLHTIVQEQQGHPTWGSYAQRLLDPEAGLWRNPSSGGHDDKAHPPIHPTKFSAGESGWSQDHHKVYELVVRHFLACVSQPAIGAVTTVDIDIAGEQFSASGTVILAKNYLDVYRFETWGGSMIPTYNYGQQFTPTTLTLDSGVTRPPPLLSEADLLSCMDNAGIGTDATMHDHIKKLLDRFYATKDSNMRFSPTKLGEALVKGYDDMGYELWKPNLRAMMESDMKAVSMGTKRKSEVLDSCLQQMKACFVDARLNKEKLFEAMDVFFERSNRANGNEQQAIGEVVRKCGLCQESDMVLRKKPDGNFMVGCLGYPQCRNVVWLPGSVSEATVTTTICSTCSPGPVYMIQFKFRRLEIPPNYNVDHLGCIGGCDDTLRQLVEICGTGSRTTSSVPGRGQGHTSSSSSAQQSNYRDQGAWQTASSAWQTASGSHPSQSSRGRSARSQRAGGAPDGESSIPCTSCGASCNLRTANTEANKGRKFYSCQAQGCSFFVWEDNINSGGTAARGGGGRSASTTSRRGGRGRGSRGGGRTNDVAFVSATGEPISGRCFVCGEPGHFSNVCPCRGR

SEQ ID NO: 43 - protein, 936 aa, Aquilegia caerula
MSRPIRVLNVAEKPSVAKSVATILSGGTNFCPSRLSHSQYNRIFEFHYTIRNQPCEMLVTSVTGHLMEIDFDDRYRKWNSCDPAILYEAPVKKFVPQDKLNVKKTLQDEAKHCQWLVLWLDCDQEGENIAFEVVDVCCAVNPRLDVWRARFSALTSRDVYQAVQNLVRPNKWLADAVDVRQESDLRVGASFTRFQTQLLTNAYLINLNNSANAHQAEGDRNHVLSYGPCQFPTLGFVVERYWEIQAHEPEEFWTINCSHTAEEGTATFSWMRGHMFDYSCAVMIYEMCVEEPTATVIKVLDQQKLKNPPFPLNTVELNKRASWYFRMSSEHTMKVAEDLYQSGFISYPRTETDSFAGNTDLHAIVQEQQEHPVWGSYAQRLLDPEAGLWKNPRIGTHSDNAHPPIYPTKFSAGESRWTQDHHRLYELVVRHFLACVSQPAIGAETKIEIDIAGELFSVSGRTIIAKNYLDVYRFESWGNSTIPKYTFGQQFVPTTLTLDSGVTRPPPLLSEADLINCMDKAGIGTDATMHDHIKKLLDRLYATKDANTRFAPTKLGEALVMGYDDMGYEELWKPSQRSRMESETKEVSVGRKSKSEVLASYLQDMKAYFLDARLNQVKLKEAMDIFFERSNRSAGDDHRAVGDTVRRCGVCNDSDMVLKRRPDGNFMVGCLGFPQCRNVVWLPGSISEATVTTQVCNSCSPGPVYMIQFKFRMLEIPPGYNVNHLGCIGGCDEILRHLTEICGTGSRNPSSVPVSSARGRGPRAPSSNAQQTSTRQGACIHCRQTGHSSSDCPSQVVQPQRAQPRRRNTQNENAGEASIPCTTCGESCVLRTANTDNNRGRKFYSCQGCNFFVWEDSMNDSAGGNTQGANRGRLTSNPRSSSARRGGRGRGSRGGRQGANTTGATFVSATGDPLSNRCFSCGDPSHFANACPNRGR

SEQ ID NO: 44 - protein, 862 aa, Setaria italica
MQPGGGGGAIRVLNVAEKPSVAKAVAEILSRGSMQSRAGRSPYNRVFEFNYAINGRACRMLVTSVTGHLMELEFDDRFRRWHSCDPADLFHAPVRKSVPQDKQAIKQTLEEEARRCQWLVLWLDCDREGENIAYEVIEVCTGANSHLNIWRARFSALIDREIHESVQHLGRPNKLFADAVDARQEIDLRIGASFTRFQTMLLKDAFVIDVTGDDRNLVLSYGPCQFPTLGFIVERFWEIQAHEPEEFWTINCTHTSDEGTASFGWIRGHLFDYPSAVILYEMCVEEPMATVQNVRNQEKLKYPPYPLSTLELQKRASRYFRMSSEHTMKVAEELYQAGFISYPRTETDNFSPNTDLHAIVREQVEHPVWGAYAHRLLTPEERLWRNPSNGGHDDKAHPPIHPTKFSRGENNWSPDHNRLYELVVRHFLACCSQPAVGAETTVEIDIAGEQFNASGRVVLAKNYLDVYRFDSWGGTLLPTYNIGQQFVPTTLTLDSGVTRPPPLLAEADLLSCMDKAGIGTDATMHDHIKKLLDRCYATKDENTRFSPTNLGEALVMGYDEMGYELWKPYLRSMMEADMKSVSIGTKSKSQVLESCLQQMKACFLDARVNKAKLLDAMGTFFARSNRPVNETQNPIEVVRPCAACRESEMVLKQKQNGEFMVGCRSYPQCRNVVWLPGSLSEASVTNQVCPICTPGPVYKIQFKFRRRDIPPNFDVDHLGCIGGCDDILKELTEISRFGSRSQAATPGQVLCTSCGELCISRIANTEANRGRKFYKCEDPGCGFFKWEDELDNATPRGRRGRGSSRQAPASAGRRGGAQARGRRGRGRNTDGGMFVSATGDPSRCCFTCGDPSHFANACPNRR

SEQ ID NO: 45 - protein, 1390 aa, Arabidopsis thaliana
  DOMAIN (129)..(272): Domaine hélicase DEXDc
  DOMAIN (445)..(570): Domaine hélicase HELICc
MGSRVPIETIEEDGEFDWEAAVKEIDLACLKTTNASSSSSSHFTPLANPPITANLTKPPAKRQSTLDKFIGRTEHKPENHQVVSECGVNDNDNSPLVGIDPEAAKTWIYPGFVPLRDYQFAITKTALFSNTLVALPTGLGKTLIAAVVMYNYFRWFPQGKIVFAAPSRPLVMQQIEACHNIVGIPQEWTIDLTGQTCPSKRAFLWKSKRVFFVTPQVLEKDIQSGTCLTNYLVCLVIDEAHRALGNYSYCVVVRELMAVPIQLRILALTATPGSKTQAIQGIIDNLQISTLEYRNESDHDVCPYVHDRKLEVIEVPLGQDADDVSKRLFHVIRPYAVRLKNFGVNLNRDIQTLSPHEVLMARDKFRQAPLPGLPHVNHGDVESCFAALITLYHIRKLLSSHGIRPAYEMLEEKLKEGPFARLMSKNEDIRMTKLLMQQRLSHGAPSPKLSKMLEILVDHFKVKDPKTSRVIIFSNFRGSVRDIMNALSNIGDMVKATEFIGQSSGKTLKGQSQKIQQAVLEKFRAGGFNVIVATSIGEEGLDIMEVDLVICFDANVSPLRMIQRMGRTGRKNNGRPLLVLACEGSEKNSYMRKQASGRAIKKHMRNGGTNSFNFHPSPRMIPHVYKPEVQHVEFSIKQFVPRGKKLQEEYATETPAFQKKLTPAETHMLAKYYNNPDEEKLRVSLIAFPHFQTLPSKVHKVMHSRQTGMLIDAMQHLQEPTFSEQSKSFFTEFRAPLGEREELDTGLRVTNDPKDLHSVRDLEVNTSQRKAKQVESPTSTLETTEKDYEESSPTHRYLFSSECASVDTLGNVFVMPVPLLFFPNVLESDNTPLPKTEKQHSCRNTSHIDLVPVDTSEKHRQDNISCKLKERFSPDGASETLETHSLVKRNSTRVGEDDVANSVGEIVLSSDEDDCEGLELSPRLTNFIKSGIVPESPVYDQGEANREEDLEFPQLSSPMRFSNELAGESSFPERKVQHKCNDYNIVSTTTELRTPQKEVGLANGTECLAVSPIPEDWRTPLANLTNTNSSARKDWRVSSGEKLETLRQPRKLKRLRRLGDCSSAVKENYPGITEADHIRSRSRGKKHIRVKWKSAESWFTLSSVAFALVTKKKKMIMDDDVQVFIDEEAEVSSGAEMSADENEDVTGDSFEDSFIDDGTMPTANTQAESGKVDMMAVYRYIQPKISFFYCEVNELIKNHKVSFHRRSLLSQSPLPARFRDLAASSLSPYSAGPLTRINESRSDSDKSLSSLRTPKTTNSESNQDAMMIGNLSVVQISSDSRKRKFSLCNSANAPVINLESKFAAHAQATEKESHEGVRSNAGALEYNDDDDDAFFATLDFDAMEAQATLLLSKQRSEAKEKEDATVIPNPGMQRSDGMEKDAPSFDLGLW

SEQ ID NO: 46 - protein, 672 aa, Arabidopsis thaliana
  DOMAIN (268)..(346): Domaine de liaison à RAD51
  DOMAIN (431)..(561): Domaine AAA
  DOMAIN (623)..(672): Domaine VPS4
MCGSVVSDSEREFEFHFWGFGHLGKEEERIMAGKRSSPFSSPLLRPPPEFLNVKEEGETETPCWRKEVDENLKRLQSLLFGADKFLEKSDFSSAQILGLRLLGFLDSRSVTDADRDFIGPIRREVASKIDLALEGLVSDSDRKAFELANTAPGAIFGSKGGFDVEKIKQSKYFGFHVSQSNGKGVKEMLIPKAPKSMMQAKLTSLYGNSIGKPDNQRKTSVNNQDRASDECVIVERSHGFGFGTKRPHAETSSLANDGEVKEDGAPNGFVSAKIKLEMDVRQKRGSTESPSSCLSPQSDKNALGRGYGSRSGGLRRGYRSNFVPPVKTNGNNVGNLTSRIGGKTDDALDDSTRTCLEMLCGPDGELPEKLRNLEPRLIEHVSNEIMDRDPNVRWDDIAGLEHAKKCVTEMVIWPLLRPDIFKGCRSPGKGLLLFGPPGTGKTMIGKAIAGEAKATFFYISASSLTSKWIGEGEKLVRALFGVASCRQPAVIFVDEIDSLLSQRKSDGEHESSRRLKTQFLIEMEGFDSGSEQILLIGATNRPQELDEAARRRLTKRLYIPLPSSEARAWIIQNLLKKDGLFTLSDDDMNIICNLTEGYSGSDMKNLVKDATMGPLREALKRGIDITNLTKDDMRLVTLQDFKDALQEVRPSVSQNELGIYENWNNQFGSLSL